European Patent Specification EP 3 464 579 B1, published July 17, 2024. Title: COMPOSITIONS COMPRISING POLYPEPTIDES HAVING GALACTANASE ACTIVITY AND POLYPEPTIDES HAVING BETA-GALACTOSIDASE ACTIVITY. Applicant: Novozymes A/S. The sequence listing filed with the application follows.

SEQUENCE LISTING (85 sequences)

SEQ ID NO: 1 - DNA, 1047 bp, Cohnella sp-60555
  CDS (1)..(1044)
  sig_peptide (1)..(96)
  mat_peptide (97)..(1044)
atgatgttcaagagaacggtaacgggcatgatggccttgctgctggtgctggctctgttcgtcgcgcaaggttcgcagccgcaccaagccgccgcggcgccgtcgttcgccaaaggggcggacatcagctgggtgccgggaatggaagcccaggggtacaagtggaaggacaagaacggcgtgcagcgggacattttggacattttgaaaaacgattatcagatcaactccgtgcgcatccgcgtgtgggtcaacccttcgagcagctacacgaacgggtacctgaacaaggaccgtgcggccgcgctggcgaagcgggccaaggcggcggggatgagcgtcatgctgacgctccattacagcgacagctgggcggaccccggccaacagacgaagccggcggcatggaagagctacacgttccagcaactgatggacgccgtgtggaactggacacgcgacgtcatgacgacgatgcaggcgaacggcgtgacgccggactgggtgcagatcggcaacgagacgaacaacggcatgctgtgggacgacggcaaggcttcgctcagcatgaagaattatgcgtggctcgtgaacacgggcaacaacgcggtgaagtcgatcagcagctcgaccaagacgatcgtgcacctggccaacggctacgacaattcgctgttcgtctggaacatcggaggcttgatcgccaacggagcgacgttcgacatcatcggcatgtcgctctatccgagcgcgtcggattggtcggccaaggtgacgcagacgatcgcgaacgcgaacgacatgatctcgcgttacggcaagccgatcatggtgacggagatcggcatggactacagccagccgagcgcggccaagagcttcgtgtcggacatcaagacgaagatccgcaacctgtccggcggcaaggggcaaggcgtgttctactgggagcccgaagcgacgcccggctacaacggcggctacagcatgggcgcctggcaagcggacatgaagccgacgatcgcgctcgagggcttctggaactaa

SEQ ID NO: 2 - protein, 348 aa, Cohnella sp-60555
MMFKRTVTGMMALLLVLALFVAQGSQPHQAAAAPSFAKGADISWVPGMEAQGYKWKDKNGVQRDILDILKNDYQINSVRIRVWVNPSSSYTNGYLNKDRAAALAKRAKAAGMSVMLTLHYSDSWADPGQQTKPAAWKSYTFQQLMDAVWNWTRDVMTTMQANGVTPDWVQIGNETNNGMLWDDGKASLSMKNYAWLVNTGNNAVKSISSSTKTIVHLANGYDNSLFVWNIGGLIANGATFDIIGMSLYPSASDWSAKVTQTIANANDMISRYGKPIMVTEIGMDYSQPSAAKSFVSDIKTKIRNLSGGKGQGVFYWEPEATPGYNGGYSMGAWQADMKPTIALEGFWN

SEQ ID NO: 3 - protein, 316 aa, Cohnella sp-60555
  mat_peptide (1)..(316)
APSFAKGADISWVPGMEAQGYKWKDKNGVQRDILDILKNDYQINSVRIRVWVNPSSSYTNGYLNKDRAAALAKRAKAAGMSVMLTLHYSDSWADPGQQTKPAAWKSYTFQQLMDAVWNWTRDVMTTMQANGVTPDWVQIGNETNNGMLWDDGKASLSMKNYAWLVNTGNNAVKSISSSTKTIVHLANGYDNSLFVWNIGGLIANGATFDIIGMSLYPSASDWSAKVTQTIANANDMISRYGKPIMVTEIGMDYSQPSAAKSFVSDIKTKIRNLSGGKGQGVFYWEPEATPGYNGGYSMGAWQADMKPTIALEGFWN

SEQ ID NO: 4 - protein, 324 aa, Artificial Sequence
  Mature sequence with His-tag
  mat_peptide (1)..(324)
HHHHHHPRAPSFAKGADISWVPGMEAQGYKWKDKNGVQRDILDILKNDYQINSVRIRVWVNPSSSYTNGYLNKDRAAALAKRAKAAGMSVMLTLHYSDSWADPGQQTKPAAWKSYTFQQLMDAVWNWTRDVMTTMQANGVTPDWVQIGNETNNGMLWDDGKASLSMKNYAWLVNTGNNAVKSISSSTKTIVHLANGYDNSLFVWNIGGLIANGATFDIIGMSLYPSASDWSAKVTQTIANANDMISRYGKPIMVTEIGMDYSQPSAAKSFVSDIKTKIRNLSGGKGQGVFYWEPEATPGYNGGYSMGAWQADMKPTIALEGFWN

SEQ ID NO: 5 - DNA, 1044 bp, Cohnella xylanilytica
  CDS (1)..(1041)
  sig_peptide (1)..(87)
  mat_peptide (88)..(1041)
atgttgcgcaaagcggttgcggtgttcatcaccttggtgttgggactgactctactatcggcgcagggaggacgaccgcaggaagcggcggcggctccgtcgttcgctaagggagcggacatcagctgggtgccgggaatggaagcgcaagggtacaggtggaaggacaagaacggcgtgcagcgggacatcctggacattctcaagaacgattaccagatcaactccgtccgcattcgggtatgggtcaatccttcgagcagctatacgaacggctacctgaacaaggaccgggcggccgcgctcgcgaagcgggcgaaggcggcggggctcagcgtcatgctgacgctgcattacagcgacagctgggccgaccccgggaagcagacgaagccggcggcgtgggccgggtacaacttccagcagctgatggacgcggtgtggaactggacgcgcgaggtcatgacgacgatgcaggccagcggggtgacgccggactgggtgcagatcggcaacgagacgaacaacggcatgctgtgggacgacgggaaggcctcgctgagcatgaagaattacgcctggctcgtcaacacgggcaacaacgcggtcaagtcgatcagcagcgggacgaaaacgatcgtgcatctcgccaacgggtacgacaattcgttgttcgtctggaacatcggcggcctgatcgcgaacggcgccacgttcgacattatcggcatgtcgctgtatccgagcgcgtccgactggtcctcgaaggtgacgcagacgatctccaacgcgaacgatatgatctcccggtacggcaagccgatcatgatcacggagatcggcatggactacaaccagccgtcggcggccaagagcttcgtcgcggatatcaagacgaagatccgcagcctgtccggcggccgagggctcggcgtcttctactgggagccggaggcgaccccgggttataacggaggctataacaagggagcctggcaggcagacatgaagccgacgatcgctctcgaaggttttctgaactaa

SEQ ID NO: 6 - protein, 347 aa, Cohnella xylanilytica
MLRKAVAVFITLVLGLTLLSAQGGRPQEAAAAPSFAKGADISWVPGMEAQGYRWKDKNGVQRDILDILKNDYQINSVRIRVWVNPSSSYTNGYLNKDRAAALAKRAKAAGLSVMLTLHYSDSWADPGKQTKPAAWAGYNFQQLMDAVWNWTREVMTTMQASGVTPDWVQIGNETNNGMLWDDGKASLSMKNYAWLVNTGNNAVKSISSGTKTIVHLANGYDNSLFVWNIGGLIANGATFDIIGMSLYPSASDWSSKVTQTISNANDMISRYGKPIMITEIGMDYNQPSAAKSFVADIKTKIRSLSGGRGLGVFYWEPEATPGYNGGYNKGAWQADMKPTIALEGFLN

SEQ ID NO: 7 - protein, 318 aa, Cohnella xylanilytica
  mat_peptide (1)..(318)
AAAPSFAKGADISWVPGMEAQGYRWKDKNGVQRDILDILKNDYQINSVRIRVWVNPSSSYTNGYLNKDRAAALAKRAKAAGLSVMLTLHYSDSWADPGKQTKPAAWAGYNFQQLMDAVWNWTREVMTTMQASGVTPDWVQIGNETNNGMLWDDGKASLSMKNYAWLVNTGNNAVKSISSGTKTIVHLANGYDNSLFVWNIGGLIANGATFDIIGMSLYPSASDWSSKVTQTISNANDMISRYGKPIMITEIGMDYNQPSAAKSFVADIKTKIRSLSGGRGLGVFYWEPEATPGYNGGYNKGAWQADMKPTIALEGFLN

SEQ ID NO: 8 - protein, 326 aa, Artificial Sequence
  Mature sequence with His-tag
  mat_peptide (1)..(326)
HHHHHHPRAAAPSFAKGADISWVPGMEAQGYRWKDKNGVQRDILDILKNDYQINSVRIRVWVNPSSSYTNGYLNKDRAAALAKRAKAAGLSVMLTLHYSDSWADPGKQTKPAAWAGYNFQQLMDAVWNWTREVMTTMQASGVTPDWVQIGNETNNGMLWDDGKASLSMKNYAWLVNTGNNAVKSISSGTKTIVHLANGYDNSLFVWNIGGLIANGATFDIIGMSLYPSASDWSSKVTQTISNANDMISRYGKPIMITEIGMDYNQPSAAKSFVADIKTKIRSLSGGRGLGVFYWEPEATPGYNGGYNKGAWQADMKPTIALEGFLN

SEQ ID NO: 9 - DNA, 1050 bp, Paenibacillus tundrae
  CDS (1)..(1047)
  sig_peptide (1)..(99)
  mat_peptide (100)..(1047)
atgttcaaaaatgtaaggggtttcaagacatccatcatgttggcttttgttttgttattcacctccatcatgttgcccgcaggtcagcatgccagcgcagcaccaagtttcgccaaaggagccgacatcagctgggttcccggaatggaagcccaaggttacaaatggaaagataaaaacggggtacagcgtgacatcattgatattttgaaaaaggactatcaaattaactccgttcgcattcgggtctttgttaatccttcgaatgattatgggaacggttacatgaataaggaacgtgcggctacactcgcacaacgtgctaaaaatgccggcatgagcgtaatgcttaccctgcattacagcgactcttgggcagaccctggtcaacagaccaaaccagctgcctggaaaaactataccttccaacagctcatggacgcagtgtggaatcacacacgtgatgtcatgactgcgatgcaaagcaaaggcgttaccccggactgggtacagatcgggaatgaaacaagtaacggcatgttatgggaagatggtaaagcatccaccaacatgaaaaactatgcgtggctggtgaacacaggccataatgcagtgaaatccctgagcagtggcaccaaaaccattgtgcacctggcaggtggggatgataacgccctctatgtatggaatattggtggtttgatcaataatggagctaactttgacatgattgccatgtccctctacccttcggcttccggctggaacacagctgtgacgaatacggtaaacaatgccaaggatatgatcaaccgttatggcaaagagatcatcatctccgaaattggcatggataataaccaggctgcagcaggtaaaagttttgttgcggcgatgaaaaaccaaatccgcaatctgccgaatggcaaaggaaaaggcgtattctactgggagcctcaggctacaccaggttataacagtggctacggcaaaggcgcttggcaatcgaatatgatgccgacagttgtcatggaaggatttattgactag

SEQ ID NO: 10 - protein, 349 aa, Paenibacillus tundrae
MFKNVRGFKTSIMLAFVLLFTSIMLPAGQHASAAPSFAKGADISWVPGMEAQGYKWKDKNGVQRDIIDILKKDYQINSVRIRVFVNPSNDYGNGYMNKERAATLAQRAKNAGMSVMLTLHYSDSWADPGQQTKPAAWKNYTFQQLMDAVWNHTRDVMTAMQSKGVTPDWVQIGNETSNGMLWEDGKASTNMKNYAWLVNTGHNAVKSLSSGTKTIVHLAGGDDNALYVWNIGGLINNGANFDMIAMSLYPSASGWNTAVTNTVNNAKDMINRYGKEIIISEIGMDNNQAAAGKSFVAAMKNQIRNLPNGKGKGVFYWEPQATPGYNSGYGKGAWQSNMMPTVVMEGFID

SEQ ID NO: 11 - protein, 316 aa, Paenibacillus tundrae
  mat_peptide (1)..(316)
APSFAKGADISWVPGMEAQGYKWKDKNGVQRDIIDILKKDYQINSVRIRVFVNPSNDYGNGYMNKERAATLAQRAKNAGMSVMLTLHYSDSWADPGQQTKPAAWKNYTFQQLMDAVWNHTRDVMTAMQSKGVTPDWVQIGNETSNGMLWEDGKASTNMKNYAWLVNTGHNAVKSLSSGTKTIVHLAGGDDNALYVWNIGGLINNGANFDMIAMSLYPSASGWNTAVTNTVNNAKDMINRYGKEIIISEIGMDNNQAAAGKSFVAAMKNQIRNLPNGKGKGVFYWEPQATPGYNSGYGKGAWQSNMMPTVVMEGFID

SEQ ID NO: 12 - protein, 324 aa, Artificial Sequence
  Mature sequence with His-tag
  mat_peptide (1)..(324)
HHHHHHPRAPSFAKGADISWVPGMEAQGYKWKDKNGVQRDIIDILKKDYQINSVRIRVFVNPSNDYGNGYMNKERAATLAQRAKNAGMSVMLTLHYSDSWADPGQQTKPAAWKNYTFQQLMDAVWNHTRDVMTAMQSKGVTPDWVQIGNETSNGMLWEDGKASTNMKNYAWLVNTGHNAVKSLSSGTKTIVHLAGGDDNALYVWNIGGLINNGANFDMIAMSLYPSASGWNTAVTNTVNNAKDMINRYGKEIIISEIGMDNNQAAAGKSFVAAMKNQIRNLPNGKGKGVFYWEPQATPGYNSGYGKGAWQSNMMPTVVMEGFID

SEQ ID NO: 13 - DNA, 1056 bp, Paenibacillus barcinonensis
  CDS (1)..(1053)
  sig_peptide (1)..(105)
  mat_peptide (106)..(1053)
atgtttaaaaatgtaaggggtttcaaggttaagacaagcgttctgctggcattggttttgttatttacttctattctgctgcctgcaggccagcacgccagcgccgcaccgagctttgccaagggagctgacatcagctgggttcccggcatggaggctcaagggtacaaatggaaggataaaaacggggtacaacgtgatattattgatattttgaaaaaggattaccaaattaactccgttcgtattcgggtattcgttaatccatcgaacgattatggtaacggttacatgaataaggatcgcgcggctgctcttgcacagcgtgccaaaaatgcaggcatgagtgtcatgctcacacttcactacagcgattcctgggcagacccaggcaaacaaagcaaaccagcggcatggaaaaattactccttccaacagctcatggacgctgtctggaattatacacgtgaagtgatgacagctatgcaaaacaaaggggttacgccggactgggtacagatcggtaacgaaacaagcaacggcatgttatgggatgacgggaaagcctctgttaacatgaaaaactatgcatggctcgtgaacacaggacataatgcggtaaaatccattagcagcggcaccaaaacgatcgttcatctggccggtggcgacgacaatgcgctgtatgtctggaatattggcggcctgatcaacaacggcgctaactttgacatgatcgctatgtcgctttacccttccgcttccggctggaatactgcggtgaccaacacggtcaacaatgcaaaggatatgatcaatcggtacggcaaagagatcatgatctccgaaattggcatggacaacaatcaggcggcggcaggcaaaagcttcgtagctgcgatgaaaaatcaaattcgcaatctgccaaatggcaaaggaaaaggcgtattctactgggagccgcaggctacacctggctataacggtggatacggtaaaggcgcttggcagtccaacatgatgccaacagccgtcatggaagggtttattgactaa

SEQ ID NO: 14 - protein, 351 aa, Paenibacillus barcinonensis
MFKNVRGFKVKTSVLLALVLLFTSILLPAGQHASAAPSFAKGADISWVPGMEAQGYKWKDKNGVQRDIIDILKKDYQINSVRIRVFVNPSNDYGNGYMNKDRAAALAQRAKNAGMSVMLTLHYSDSWADPGKQSKPAAWKNYSFQQLMDAVWNYTREVMTAMQNKGVTPDWVQIGNETSNGMLWDDGKASVNMKNYAWLVNTGHNAVKSISSGTKTIVHLAGGDDNALYVWNIGGLINNGANFDMIAMSLYPSASGWNTAVTNTVNNAKDMINRYGKEIMISEIGMDNNQAAAGKSFVAAMKNQIRNLPNGKGKGVFYWEPQATPGYNGGYGKGAWQSNMMPTAVMEGFID

SEQ ID NO: 15 - protein, 316 aa, Paenibacillus barcinonensis
APSFAKGADISWVPGMEAQGYKWKDKNGVQRDIIDILKKDYQINSVRIRVFVNPSNDYGNGYMNKDRAAALAQRAKNAGMSVMLTLHYSDSWADPGKQSKPAAWKNYSFQQLMDAVWNYTREVMTAMQNKGVTPDWVQIGNETSNGMLWDDGKASVNMKNYAWLVNTGHNAVKSISSGTKTIVHLAGGDDNALYVWNIGGLINNGANFDMIAMSLYPSASGWNTAVTNTVNNAKDMINRYGKEIMISEIGMDNNQAAAGKSFVAAMKNQIRNLPNGKGKGVFYWEPQATPGYNGGYGKGAWQSNMMPTAVMEGFID

SEQ ID NO: 16 - protein, 324 aa, Artificial Sequence
  Mature sequence with His-tag
  mat_peptide (1)..(324)
HHHHHHPRAPSFAKGADISWVPGMEAQGYKWKDKNGVQRDIIDILKKDYQINSVRIRVFVNPSNDYGNGYMNKDRAAALAQRAKNAGMSVMLTLHYSDSWADPGKQSKPAAWKNYSFQQLMDAVWNYTREVMTAMQNKGVTPDWVQIGNETSNGMLWDDGKASVNMKNYAWLVNTGHNAVKSISSGTKTIVHLAGGDDNALYVWNIGGLINNGANFDMIAMSLYPSASGWNTAVTNTVNNAKDMINRYGKEIMISEIGMDNNQAAAGKSFVAAMKNQIRNLPNGKGKGVFYWEPQATPGYNGGYGKGAWQSNMMPTAVMEGFID

SEQ ID NO: 17 - DNA, 1044 bp, Paenibacillus sp-62603
  CDS (1)..(1041)
  sig_peptide (1)..(93)
  mat_peptide (94)..(1041)
atgaaacgaaggttttacagtttgacgcttgttgtcgccttgttaatgactatttttggagtgaatgggggatctgtgccgcaggtcagcgcagctcctgcattcgcgaaaggtgcggacattagctgggtagtcggcatggaggcgcaagggtatacgtggaaggacaaaaacggcgtaactagggacattattcaaattttgaagcaggattaccaaatcaactccgtacgtattcgagtattcgtcaatccttcttcgaactatggcaacgggtatatgaataaagatcgcgctgcaaccttggcgaagcgggcgaaggatgctgggatgagcgtcatgcttacattgcattacagcgattcgtgggcggaccccggaaaacagacaaagccagcggcttgggcaagctattcgttccagcagctgatggatgcagtttataatcatacgcgtgaggtaatgacagctatgcaaagcaaaggtgtcacaccggattgggtgcaaatcggcaacgaaacgaacgatggcatgctctggaatgacgggaaagcttccttaaacatgcaaaactacgcttggctgatcaacactggcaacaatgcggtcaagtccattagttcagctacaaaaacgattgtccacttgtccaacggttatgacaacagtttatttgtctggaatatcggcggactgatcgctaacggagcgaccttcgatattatcgggatgtcactttatcctaccagtgctgattggtcgactaaggttacgcaaacggtcagcaactccaacaatatgatatcgcgttatggcaagccggttatgattaccgaaattggtatggattataaccagcctgccgctgccaaaagctttgtcgctgatataaagacaaaaatacgtaatattgcaggtggaaaagggcttggcgtgttttattgggaaccggaagcgacccctggttataacggaggttataataagggagcttggcaggcggacggcaaaccaacaattgcgcttgacggcttcttgaattaa

SEQ ID NO: 18 - protein, 347 aa, Paenibacillus sp-62603
MKRRFYSLTLVVALLMTIFGVNGGSVPQVSAAPAFAKGADISWVVGMEAQGYTWKDKNGVTRDIIQILKQDYQINSVRIRVFVNPSSNYGNGYMNKDRAATLAKRAKDAGMSVMLTLHYSDSWADPGKQTKPAAWASYSFQQLMDAVYNHTREVMTAMQSKGVTPDWVQIGNETNDGMLWNDGKASLNMQNYAWLINTGNNAVKSISSATKTIVHLSNGYDNSLFVWNIGGLIANGATFDIIGMSLYPTSADWSTKVTQTVSNSNNMISRYGKPVMITEIGMDYNQPAAAKSFVADIKTKIRNIAGGKGLGVFYWEPEATPGYNGGYNKGAWQADGKPTIALDGFLN

SEQ ID NO: 19 - protein, 316 aa, Paenibacillus sp-62603
  mat_peptide (1)..(316)
APAFAKGADISWVVGMEAQGYTWKDKNGVTRDIIQILKQDYQINSVRIRVFVNPSSNYGNGYMNKDRAATLAKRAKDAGMSVMLTLHYSDSWADPGKQTKPAAWASYSFQQLMDAVYNHTREVMTAMQSKGVTPDWVQIGNETNDGMLWNDGKASLNMQNYAWLINTGNNAVKSISSATKTIVHLSNGYDNSLFVWNIGGLIANGATFDIIGMSLYPTSADWSTKVTQTVSNSNNMISRYGKPVMITEIGMDYNQPAAAKSFVADIKTKIRNIAGGKGLGVFYWEPEATPGYNGGYNKGAWQADGKPTIALDGFLN

SEQ ID NO: 20 - protein, 324 aa, Artificial Sequence
  Mature sequence with His-tag
  mat_peptide (1)..(324)
HHHHHHPRAPAFAKGADISWVVGMEAQGYTWKDKNGVTRDIIQILKQDYQINSVRIRVFVNPSSNYGNGYMNKDRAATLAKRAKDAGMSVMLTLHYSDSWADPGKQTKPAAWASYSFQQLMDAVYNHTREVMTAMQSKGVTPDWVQIGNETNDGMLWNDGKASLNMQNYAWLINTGNNAVKSISSATKTIVHLSNGYDNSLFVWNIGGLIANGATFDIIGMSLYPTSADWSTKVTQTVSNSNNMISRYGKPVMITEIGMDYNQPAAAKSFVADIKTKIRNIAGGKGLGVFYWEPEATPGYNGGYNKGAWQADGKPTIALDGFLN

SEQ ID NO: 21 - DNA, 1050 bp, Paenibacillus xylanilyticus
  CDS (1)..(1047)
  sig_peptide (1)..(99)
  mat_peptide (100)..(1047)
atgcttaaatttgtaaggggttacaaaacatcgattgctcttgttcttgtgttgttgttcacctccattatgctgcctgtgggtcagcatgtcagcgcagcacccagcttcgccaagggggctgatataagctgggtaccaggcatggaagcgcaagggtacaaatggaaagacaaaaatggtgtacagcgtgacattattgatattttgaaaaacgattatcagatcaactcggttcgtatccgggtgtttgttaatccttctaatgattacggcaacgggtacatgaataaggatcgtgtcgctgctttggcacagcgggccaaaaacgcgggcatgagcgtcatgttgactctgcactacagtgattcctgggcagaccctggccaacagaccaaaccggcagcctggaaaaactacaccttccagcagctgatggatgccgtttggaatcatacacgcgatgtgatgacggccatgcagagtaaaggggttacgcctgactgggtacaaatcgggaacgaaacaagcaacggcatgttatgggaggacggtaaagcgtccacgaacatgaaaaattacgcatggctggtgaacacgggccataatgccgtcaagtccatgagtacagggaccaaaacgattgtccatcttgcaggcggtgacgacaatgccctttatgtatggaatatcggcggactgatcaacaacggtgccaacttcgatatgattgccatgtccctctatccttcggcttccggctggaatacagctgtcaccaatacggtgaataatgccaaggacttgatcaaccgctacggcaaagagattatcgtctcagaaatcggcatggacaacaatcagcccgcagctggcaaaagtttcgttgctgcgatgaaaaatcaattccgcaacctgccaaatgggaaaggaaaaggcgtattctactgggagccgcaggctacaccaggttataacggtggttacggcaaaggcgcttggcagtcgaatatgatgccaacagcggtcatggaaggatttatagactag

SEQ ID NO: 22 - protein, 349 aa, Paenibacillus xylanilyticus
MLKFVRGYKTSIALVLVLLFTSIMLPVGQHVSAAPSFAKGADISWVPGMEAQGYKWKDKNGVQRDIIDILKNDYQINSVRIRVFVNPSNDYGNGYMNKDRVAALAQRAKNAGMSVMLTLHYSDSWADPGQQTKPAAWKNYTFQQLMDAVWNHTRDVMTAMQSKGVTPDWVQIGNETSNGMLWEDGKASTNMKNYAWLVNTGHNAVKSMSTGTKTIVHLAGGDDNALYVWNIGGLINNGANFDMIAMSLYPSASGWNTAVTNTVNNAKDLINRYGKEIIVSEIGMDNNQPAAGKSFVAAMKNQFRNLPNGKGKGVFYWEPQATPGYNGGYGKGAWQSNMMPTAVMEGFID

SEQ ID NO: 23 - protein, 316 aa, Paenibacillus xylanilyticus
  mat_peptide (1)..(316)
APSFAKGADISWVPGMEAQGYKWKDKNGVQRDIIDILKNDYQINSVRIRVFVNPSNDYGNGYMNKDRVAALAQRAKNAGMSVMLTLHYSDSWADPGQQTKPAAWKNYTFQQLMDAVWNHTRDVMTAMQSKGVTPDWVQIGNETSNGMLWEDGKASTNMKNYAWLVNTGHNAVKSMSTGTKTIVHLAGGDDNALYVWNIGGLINNGANFDMIAMSLYPSASGWNTAVTNTVNNAKDLINRYGKEIIVSEIGMDNNQPAAGKSFVAAMKNQFRNLPNGKGKGVFYWEPQATPGYNGGYGKGAWQSNMMPTAVMEGFID

SEQ ID NO: 24 - protein, 324 aa, Artificial Sequence
  Mature sequence with His-tag
  mat_peptide (1)..(324)
HHHHHHPRAPSFAKGADISWVPGMEAQGYKWKDKNGVQRDIIDILKNDYQINSVRIRVFVNPSNDYGNGYMNKDRVAALAQRAKNAGMSVMLTLHYSDSWADPGQQTKPAAWKNYTFQQLMDAVWNHTRDVMTAMQSKGVTPDWVQIGNETSNGMLWEDGKASTNMKNYAWLVNTGHNAVKSMSTGTKTIVHLAGGDDNALYVWNIGGLINNGANFDMIAMSLYPSASGWNTAVTNTVNNAKDLINRYGKEIIVSEIGMDNNQPAAGKSFVAAMKNQFRNLPNGKGKGVFYWEPQATPGYNGGYGKGAWQSNMMPTAVMEGFID

SEQ ID NO: 25 - DNA, 1638 bp, Paenibacillus sp-18179
  CDS (1)..(1635)
  misc_feature (1)..(3): The gene has an alternative start codon gtg which would normally code for Val but is translated to Met when it is the first codon.
  sig_peptide (1)..(87)
  mat_peptide (88)..(1635)
gtgggtaaatgggttagagctattgctttagcaggtgtagttgcactttttacatctatgatcactcctcttcaagaaacaaaggctgctggaggcttcgttatggggggagacgtttcaatgctccatgaagttgagcagttaggcgggaagttttacgatcagggcactccaaaggatgctttgcaaattttaagcgcacatggcatgaatgctgtccgattgcgtctatgggttgacccgtatgacagtttcggaaatccttatggcggtggaacaaacgatctggctacgactatatctcttgcacagcgagcgaaggcacaaggtatggaggtgctgctggattttcacttcagtgatttctgggcagacccagggaagcagaacaagcctaaagcttggcagagcttaacgtacaaccagctgcttactacggtatatgattatacgcatagtgtaattacgcaaatgaaagcggctggcgtgatgcctgatatggttcaggtaggaaacgaggcaagcagcggcatcctctggaatgatggcaaggtggggggaggcattgatgattttacgaaactcggagaactgtttacctctgctattaatgggattaatgcggccctcagctctagtgagaacattgagattgttctgcatttggatcatggcggcgacaacaatttatacacttggtggttcgataaaattgaagcggagaacgtggattacgatattatcggcttgacctactatccgttttggcatggaacgatgggagaattggcgtataatcttaatgcgatcagcagtcgttacaataaggacgtaatgattgtggaaacgtcgtatggctttacgctggatgatggtgatggtttaggcaactctttttacacggcggaagaaagcattgggggttacccggctacagtagaaggccagacggcgtatttgcgggatttgaaggaaattgttagggatgtcccaaacaaccgcggccgcggcattttctggtgggagccgacatggctgcctgttgcaggggctaactgggggacggatgcaggcaagctgtacaacaatgatactggactactatctaatccttgggacaatcagaccttgtttgattttaatggaaatgtgttgtctacagtttcagtatttacacaaagtgctccaaccaaccttgttgctaatcatagctttgaggccgatggttggacaacaacaccatctagctggaatcgctgggcagccgatacggcatcctataatgctattaaggttgaagaaaacggtattacgggcagctataagctgacgcattggagtgattctgcttatgaggcctctacgtaccagactgtttcaggattaagcaatggtacctatactttatccgcttgggtgcttaacagtggcggacaaaatacgctgcagctttacgctaaaaattacgggggttcagaacggaacgtcaatcttcctgttagcccaacaaagtgggtaaaagtaaaaattgaaaacatcagtgttacaaatggtcaaatcgaattaggcatttattcagatgcgaatgctgataattggatgaacctcgataacgtcaaactttataaaacaaactag

SEQ ID NO: 26 - protein, 545 aa, Paenibacillus sp-18179
VGKWVRAIALAGVVALFTSMITPLQETKAAGGFVMGGDVSMLHEVEQLGGKFYDQGTPKDALQILSAHGMNAVRLRLWVDPYDSFGNPYGGGTNDLATTISLAQRAKAQGMEVLLDFHFSDFWADPGKQNKPKAWQSLTYNQLLTTVYDYTHSVITQMKAAGVMPDMVQVGNEASSGILWNDGKVGGGIDDFTKLGELFTSAINGINAALSSSENIEIVLHLDHGGDNNLYTWWFDKIEAENVDYDIIGLTYYPFWHGTMGELAYNLNAISSRYNKDVMIVETSYGFTLDDGDGLGNSFYTAEESIGGYPATVEGQTAYLRDLKEIVRDVPNNRGRGIFWWEPTWLPVAGANWGTDAGKLYNNDTGLLSNPWDNQTLFDFNGNVLSTVSVFTQSAPTNLVANHSFEADGWTTTPSSWNRWAADTASYNAIKVEENGITGSYKLTHWSDSAYEASTYQTVSGLSNGTYTLSAWVLNSGGQNTLQLYAKNYGGSERNVNLPVSPTKWVKVKIENISVTNGQIELGIYSDANADNWMNLDNVKLYKTN

SEQ ID NO: 27 - protein, 516 aa, Paenibacillus sp-18179
  mat_peptide (1)..(516)
AGGFVMGGDVSMLHEVEQLGGKFYDQGTPKDALQILSAHGMNAVRLRLWVDPYDSFGNPYGGGTNDLATTISLAQRAKAQGMEVLLDFHFSDFWADPGKQNKPKAWQSLTYNQLLTTVYDYTHSVITQMKAAGVMPDMVQVGNEASSGILWNDGKVGGGIDDFTKLGELFTSAINGINAALSSSENIEIVLHLDHGGDNNLYTWWFDKIEAENVDYDIIGLTYYPFWHGTMGELAYNLNAISSRYNKDVMIVETSYGFTLDDGDGLGNSFYTAEESIGGYPATVEGQTAYLRDLKEIVRDVPNNRGRGIFWWEPTWLPVAGANWGTDAGKLYNNDTGLLSNPWDNQTLFDFNGNVLSTVSVFTQSAPTNLVANHSFEADGWTTTPSSWNRWAADTASYNAIKVEENGITGSYKLTHWSDSAYEASTYQTVSGLSNGTYTLSAWVLNSGGQNTLQLYAKNYGGSERNVNLPVSPTKWVKVKIENISVTNGQIELGIYSDANADNWMNLDNVKLYKTN

SEQ ID NO: 28 - protein, 524 aa, Artificial Sequence
  Mature sequence with His-tag
  mat_peptide (1)..(524)
HHHHHHPRAGGFVMGGDVSMLHEVEQLGGKFYDQGTPKDALQILSAHGMNAVRLRLWVDPYDSFGNPYGGGTNDLATTISLAQRAKAQGMEVLLDFHFSDFWADPGKQNKPKAWQSLTYNQLLTTVYDYTHSVITQMKAAGVMPDMVQVGNEASSGILWNDGKVGGGIDDFTKLGELFTSAINGINAALSSSENIEIVLHLDHGGDNNLYTWWFDKIEAENVDYDIIGLTYYPFWHGTMGELAYNLNAISSRYNKDVMIVETSYGFTLDDGDGLGNSFYTAEESIGGYPATVEGQTAYLRDLKEIVRDVPNNRGRGIFWWEPTWLPVAGANWGTDAGKLYNNDTGLLSNPWDNQTLFDFNGNVLSTVSVFTQSAPTNLVANHSFEADGWTTTPSSWNRWAADTASYNAIKVEENGITGSYKLTHWSDSAYEASTYQTVSGLSNGTYTLSAWVLNSGGQNTLQLYAKNYGGSERNVNLPVSPTKWVKVKIENISVTNGQIELGIYSDANADNWMNLDNVKLYKTN

SEQ ID NO: 29 - DNA, 1053 bp, Paenibacillus peoriae
  CDS (1)..(1050)
  sig_peptide (1)..(99)
  mat_peptide (100)..(1050)
atgaaaacaggtaaccgcacgatggtatttgcgatgttgatcttgctttccagcttattgtatccgttcggctctgtagggttgggtgcggcttcggccgcccctgctttcgccaaaggagcagatataagctgggtagcaggaatggaagcgcaaggtatgacttggaaggataaaaagggtgttcgtcgagatatactgcaaattttgcgagatgactatcagatcaactcggtacgtatccgtgtgtgggtaaaccccgacatgaaagattatgcaagcggatacatgaatgccgaaaaggcagcagaactggcgcagcgagctaaaaaattgggtatgagcgttatgctgactctacattatagtgattcctgggcagatccagggcaacagaacaaaccttatgcgtggcgcaattttacatttacacaactcatggatgcagtctggtctcatacggtttatgttatgaacacgatgaaaagcaagggggtaacaccggactgggtgcagatcggtaatgagacgaacaatggaatgctctgggaagacggcaaagcttcggtgaacatgaaaaactatgcctggctcgtcaatacaggtaataatgctgtaaaatcggtaagcagcagtactaaaacgatagtacatttagccaacggggataacggttccgtgttgaactggaatatcggcggactgattgataatggagctcagtttgatctcatcgggctgtctctgtatccgtctccttctgactggcagggcaaggtggatcagacgattacgaatgccaataacctcattgccaaatacggtaaaggtattgtcatcagtgaaatcgggatggaatataacgaacctgcagcttccaaggcatttatttctgcaatcaaaacaaaggttcggaacatgggaggcggcaaaggcacaggggtattttattgggagccggctgcaactccaggttacaatcaaggttataacaaaggtgcttggcaggctgacggtaaaccaacctcagctttggagggatttgtaaattaa

SEQ ID NO: 30 - protein, 350 aa, Paenibacillus peoriae
MKTGNRTMVFAMLILLSSLLYPFGSVGLGAASAAPAFAKGADISWVAGMEAQGMTWKDKKGVRRDILQILRDDYQINSVRIRVWVNPDMKDYASGYMNAEKAAELAQRAKKLGMSVMLTLHYSDSWADPGQQNKPYAWRNFTFTQLMDAVWSHTVYVMNTMKSKGVTPDWVQIGNETNNGMLWEDGKASVNMKNYAWLVNTGNNAVKSVSSSTKTIVHLANGDNGSVLNWNIGGLIDNGAQFDLIGLSLYPSPSDWQGKVDQTITNANNLIAKYGKGIVISEIGMEYNEPAASKAFISAIKTKVRNMGGGKGTGVFYWEPAATPGYNQGYNKGAWQADGKPTSALEGFVN

SEQ ID NO: 31 - protein, 317 aa, Paenibacillus peoriae
  mat_peptide (1)..(317)
APAFAKGADISWVAGMEAQGMTWKDKKGVRRDILQILRDDYQINSVRIRVWVNPDMKDYASGYMNAEKAAELAQRAKKLGMSVMLTLHYSDSWADPGQQNKPYAWRNFTFTQLMDAVWSHTVYVMNTMKSKGVTPDWVQIGNETNNGMLWEDGKASVNMKNYAWLVNTGNNAVKSVSSSTKTIVHLANGDNGSVLNWNIGGLIDNGAQFDLIGLSLYPSPSDWQGKVDQTITNANNLIAKYGKGIVISEIGMEYNEPAASKAFISAIKTKVRNMGGGKGTGVFYWEPAATPGYNQGYNKGAWQADGKPTSALEGFVN

SEQ ID NO: 32 - protein, 325 aa, Artificial Sequence
  Mature sequence with His-tag
  mat_peptide (1)..(325)
HHHHHHPRAPAFAKGADISWVAGMEAQGMTWKDKKGVRRDILQILRDDYQINSVRIRVWVNPDMKDYASGYMNAEKAAELAQRAKKLGMSVMLTLHYSDSWADPGQQNKPYAWRNFTFTQLMDAVWSHTVYVMNTMKSKGVTPDWVQIGNETNNGMLWEDGKASVNMKNYAWLVNTGNNAVKSVSSSTKTIVHLANGDNGSVLNWNIGGLIDNGAQFDLIGLSLYPSPSDWQGKVDQTITNANNLIAKYGKGIVISEIGMEYNEPAASKAFISAIKTKVRNMGGGKGTGVFYWEPAATPGYNQGYNKGAWQADGKPTSALEGFVN

SEQ ID NO: 33 - DNA, 1050 bp, Paenibacillus xylanexedens
  CDS (1)..(1047)
  sig_peptide (1)..(99)
  mat_peptide (100)..(1047)
atgttcaaaaatgtaaggggtttcaggatatccatcatgttggcttttgttttgttattcacctccatcatgttgcccgcaggtcagcatgccagcgcagcaccaagtttcgccaaaggagccgacatcagttgggttcccggaatggaagctcaaggctacaaatggaaagataaaaacggggtacagcgtgacatcattgatattttgaaaaatgactatcaaatcaattccgttcgtattcgggtctttgttaatccttcgaacgattatgggaacggttacatgaacaaggatcgtgcggctgcactcgcacaacgtgccaagaatgccggcatgagcgtaatgctcaccctgcactacagcgattcctgggcagaccctggtcaacagaccaaaccagctgcctggaaaaactacacgttccagcagctcatggatgcggtgtggaatcacacacgtgatgtcatgactgcaatgcaaagcaaaggcgttaccccggactgggtacagatcgggaatgaaacaagcaacggcatgttatgggaagatggcaaagcatctaccaacatgaaaaactatgcgtggctggtaaacacaggccataatgcagtgaaatccctgagcagcggcaccaaaaccattgtgcatctggcaggtggagatgataacgccctctatgtatggaatattggaggcctgatcaataacggagccaactttgacatgattgcgatgtccctctacccttcggcttccggctggaacacagctgtgacgaatacagtaaacaatgccaaggatatgatcaaccgttatggcaaagagatcattatctccgaaattggtatggacaataaccaggctgcagctggtaaaagttttgttgcggcgatgaaaaaccaaatccgcaatctgccgaatggtaaaggcaaaggcgtattctactgggagcctcaggctacaccaggatacaacagcggctatggcaaaggtgcatggcaatcgaatatgatgccgacggtagtcatggaaggatttattgactag

SEQ ID NO: 34 - protein, 349 aa, Paenibacillus xylanexedens
MFKNVRGFRISIMLAFVLLFTSIMLPAGQHASAAPSFAKGADISWVPGMEAQGYKWKDKNGVQRDIIDILKNDYQINSVRIRVFVNPSNDYGNGYMNKDRAAALAQRAKNAGMSVMLTLHYSDSWADPGQQTKPAAWKNYTFQQLMDAVWNHTRDVMTAMQSKGVTPDWVQIGNETSNGMLWEDGKASTNMKNYAWLVNTGHNAVKSLSSGTKTIVHLAGGDDNALYVWNIGGLINNGANFDMIAMSLYPSASGWNTAVTNTVNNAKDMINRYGKEIIISEIGMDNNQAAAGKSFVAAMKNQIRNLPNGKGKGVFYWEPQATPGYNSGYGKGAWQSNMMPTVVMEGFID

SEQ ID NO: 35 - protein, 316 aa, Paenibacillus xylanexedens
  mat_peptide (1)..(316)
APSFAKGADISWVPGMEAQGYKWKDKNGVQRDIIDILKNDYQINSVRIRVFVNPSNDYGNGYMNKDRAAALAQRAKNAGMSVMLTLHYSDSWADPGQQTKPAAWKNYTFQQLMDAVWNHTRDVMTAMQSKGVTPDWVQIGNETSNGMLWEDGKASTNMKNYAWLVNTGHNAVKSLSSGTKTIVHLAGGDDNALYVWNIGGLINNGANFDMIAMSLYPSASGWNTAVTNTVNNAKDMINRYGKEIIISEIGMDNNQAAAGKSFVAAMKNQIRNLPNGKGKGVFYWEPQATPGYNSGYGKGAWQSNMMPTVVMEGFID

SEQ ID NO: 36 - protein, 324 aa, Artificial Sequence
  Mature sequence with His-tag
  mat_peptide (1)..(324)
HHHHHHPRAPSFAKGADISWVPGMEAQGYKWKDKNGVQRDIIDILKNDYQINSVRIRVFVNPSNDYGNGYMNKDRAAALAQRAKNAGMSVMLTLHYSDSWADPGQQTKPAAWKNYTFQQLMDAVWNHTRDVMTAMQSKGVTPDWVQIGNETSNGMLWEDGKASTNMKNYAWLVNTGHNAVKSLSSGTKTIVHLAGGDDNALYVWNIGGLINNGANFDMIAMSLYPSASGWNTAVTNTVNNAKDMINRYGKEIIISEIGMDNNQAAAGKSFVAAMKNQIRNLPNGKGKGVFYWEPQATPGYNSGYGKGAWQSNMMPTVVMEGFID

SEQ ID NO: 37 - DNA, 1044 bp, Cohnella laeviribosi
  CDS (1)..(1041)
  sig_peptide (1)..(93)
  mat_peptide (94)..(1041)
atgaaaagaaaaacgttcggatggctgttgacggcgctgctcggtttgaccctggcgctcggcaacgccgtgtctcccggcgacgcgaaagccgccccggcatttgcgaaaggcgcggacatcagctgggttccgggcatggaggcgcaagggtacaaatggaaggacaaaaacggcgtgcagcgggacatcattgatattttaaagcaggattaccagatcaactccgtccggatccgcgtgtttgtcaatccgtcaagcgattacggcaacggctacttgaacaaggaacgcgcggccgacttggcccagcgggcgaaaaacgccggcatgagcgtcatgctgacgctgcactacagcgattcgtgggcggaccccggcaagcaaaccaagccggccgcgtggcaaaattatacgttcgagcaattgatggacgccgtatggaactggacgcgcgatgtgatgacgacgatgcagagcagaggcgttacgccggactgggtgcagatcggcaacgagacgaacaacggcatgctgtgggatgacggcaaggcgtccgtcaacatgcgtaattacgcctggctcgtcaataccggcaacaatgcggtcaagtcgatcagcagctccacgaagacgatcgtccatctttccaacggctacgacaattcgctgttcgtctggaacatcggtgggctgatcagcaacggcgcgacgtttgacattatcggcatgtcgctgtacccgtccgcgtccgactggcagacgaaggtcaatcagacgatcagcaacgcgaacgatctgatttcgcgctacggcaagagcatcatgatctccgaaatcggcatggactacaaccagccttcggccgcgaagagcttcatctccgacatcaagacgaaggtccggaatctttccggaggcaaagggcttggcgtgttttattgggagcccgaggctacccccggctacaacggcggctacaacaagggcgcctggcagtccgacatgaagccgacgatcgcgctggaaggcttcctgaactga

SEQ ID NO: 38 - protein, 347 aa, Cohnella laeviribosi
MKRKTFGWLLTALLGLTLALGNAVSPGDAKAAPAFAKGADISWVPGMEAQGYKWKDKNGVQRDIIDILKQDYQINSVRIRVFVNPSSDYGNGYLNKERAADLAQRAKNAGMSVMLTLHYSDSWADPGKQTKPAAWQNYTFEQLMDAVWNWTRDVMTTMQSRGVTPDWVQIGNETNNGMLWDDGKASVNMRNYAWLVNTGNNAVKSISSSTKTIVHLSNGYDNSLFVWNIGGLISNGATFDIIGMSLYPSASDWQTKVNQTISNANDLISRYGKSIMISEIGMDYNQPSAAKSFISDIKTKVRNLSGGKGLGVFYWEPEATPGYNGGYNKGAWQSDMKPTIALEGFLN

SEQ ID NO: 39 - protein, 316 aa, Cohnella laeviribosi
  mat_peptide (1)..(316)
APAFAKGADISWVPGMEAQGYKWKDKNGVQRDIIDILKQDYQINSVRIRVFVNPSSDYGNGYLNKERAADLAQRAKNAGMSVMLTLHYSDSWADPGKQTKPAAWQNYTFEQLMDAVWNWTRDVMTTMQSRGVTPDWVQIGNETNNGMLWDDGKASVNMRNYAWLVNTGNNAVKSISSSTKTIVHLSNGYDNSLFVWNIGGLISNGATFDIIGMSLYPSASDWQTKVNQTISNANDLISRYGKSIMISEIGMDYNQPSAAKSFISDIKTKVRNLSGGKGLGVFYWEPEATPGYNGGYNKGAWQSDMKPTIALEGFLN

SEQ ID NO: 40 - protein, 324 aa, Artificial Sequence
  Mature sequence with His-tag
  mat_peptide (1)..(324)
HHHHHHPRAPAFAKGADISWVPGMEAQGYKWKDKNGVQRDIIDILKQDYQINSVRIRVFVNPSSDYGNGYLNKERAADLAQRAKNAGMSVMLTLHYSDSWADPGKQTKPAAWQNYTFEQLMDAVWNWTRDVMTTMQSRGVTPDWVQIGNETNNGMLWDDGKASVNMRNYAWLVNTGNNAVKSISSSTKTIVHLSNGYDNSLFVWNIGGLISNGATFDIIGMSLYPSASDWQTKVNQTISNANDLISRYGKSIMISEIGMDYNQPSAAKSFISDIKTKVRNLSGGKGLGVFYWEPEATPGYNGGYNKGAWQSDMKPTIALEGFLN

SEQ ID NO: 41 - DNA, 3352 bp, Hamigera paravellanea
  CDS (1)..(801)
  sig_peptide (1)..(69)
  mat_peptide (70)..(3349)
  CDS (873)..(1869)
  CDS (1930)..(2223)
  CDS (2297)..(2368)
  CDS (2427)..(2514)
  CDS (2578)..(3349)
atgacgcgccttagtgagtgggctttcgtcctactctcaactttgggcgtcttcgcggctgctcaggcccaaacagtgtcgcaatggcccatccacgacaatgacttgaacacagtcgtccagtgggaccactacagcttcatcattaacggacagcgtatcttcgttttctcgggcgaattccactactggcgcattccggtccccgggttatggagggatatcctcgagaaggtcaaagcggccggattcactgcgtttgcattctactccagctgggcgtaccacgctccgaataaccacaccgtcgacttctcgacaggtgcccgtgatatcacgccgatctttgacctggccaaggagcttggtttgtacgtcatcgtccgtccggggccctacgtcaacgcggaagccaatgctggtggctaccctctttggctcaccaccggtgcttatggaagcctgaggaacaatgacacgcggtacatcaatgccttggaaccttacttttccaaggtgtcgcagatcacaagccagtatcagatcaccaacgaccacaacaccatctgctatcaaatcgagaacgagtatggccagcaatggatcggcagtgcatacgacagggttccgaatgagacggccattgcatacatggaaatcctcaaggcgagcgctcgcagaaatggcattgatattcctctcacggcgaatgacccgaacatgaacactcgttcgtgggggaaagactggtccgacgaaggtggaaacgtggacatccccggcgtcgactcctatccttcggtatgtggagactatgatcattttggaggtgaaccttttctgatgtttttttcttcatctccgtcttccagtgctggtcatgcgacctcagtgtatgcacttcgacaaacggagtatacgtcccgttccaggtcctgaactactacgactatttcgcagaaacgtcaccgacgatgccgtcattcatgccagaatttcagggtggctcttacaatccctggggcggtcccgaaggtggctgtccggacgacataggaccggaatttgcgaacctgttctacaggtggaacatcggtcagcgtgtcacggctatgagtttgtatatgctctatggaggaacaaactggggtgcaatggctgctcccgtgacagctagcagctatgactattctgctcccatctcagaggatcgctccatcggcgcgaaatactatgagaccaagctcctggggctgttcagtcggagcgcgcgagacctgaccgtgacggatctgatcggcaatggaacccagtataccaacaacgtgatgattcaggcacgcgaactcagaaacccggaaaccaatgccgctttctacgtcacagttcataccaacacctctgtttctactaacgaggtcttccacctgagagtcaacacctctgccggagctctaacgattcctaaacacgcgcttggcattcgactgaatggtcaccagtcgaagatcatagtgacggactttaccttcggccccaggactctgctctactcgaccgcagaagtcctcgcctatgccgcgctggacgacaccccaactctggctctctgggttccacctggagagtccggagagtttaacgtcaagggcgcaaaatcgggatcggtcaagaaatgccaggggtgttcgaacgtccagttccaccaggaaaacggtggtcttacagtcgccttcactcaatctcaagggatgagcgttgtggaactgaacgatggtagtcgcgtggttctgcttgacagggaatccgcataccgtttctgggctccagcattgactaacgatccattcgtgccggaggatgagactggtgcgtgttttccttatgccaatcgtgaaaaaaaaaaatgcttgctgacctgccaagcagttctgatccaaggcccctacctcgtccgcggggctaaactgtcaggctctacgctgtcggtaacaggtgatatcgtgaatgcaacgaccgtggagatcttcgcgcccaaaaccgtcaagtccattacctggaacgggagagaactgaagacttcgaagacgtcttatggcagtctgcagggctctttgaaggctcctgcacccgtcaaattgcccgctcttaccggctggaaatccaaggacagcttgcccgagcggcttgcatcatatgacgactctggtgcggcctgggttggtgagtagaagaaaatcataagcagttgaacggagcggaatagaacagaatcggtaaactgacatccaccaagatgccaaccacatgacaacattgaacccgagccctccagcaacacttccagtcctatacgccgacgaatatggtattgccgcctcctttccacctgtttccgacgatccgtcatactgactttcgtataggcttccacaacggcgtccgtctctggcgaggctacttcaacggcaccgctacgggggtcttcttgaacatccaaggaggaagcgccttgtaagctattcacaatcgccactcagcaaagcccgggtccaatactaacatctcgacacacagcggctggtcagcctacctcaacggccacttcctgggatcccatctcggcgccgcctccatcgcccaagccaaccgtaccctctccttcgccaacgccaccctcaatgcctttggccccaatgtcctcctcgtcatccacgacgacacaggccacgatcaaaccaccggtgccctgaacccgcgcggcattctgaacgcgaccctcctctccggcgacgactcggcccaattcactcactggcgcctcgccggcaccgccggcggcgaatccaacctcgaccccgtccgcggcgtgtacaacgaagacggcctcttcgccgagcgcgtcggctggcacctccccgggttcgacgactcggcttggcccgacgcctcgtctccgcgcgagggcttcgcgggcgcgaccgtccggttctaccggaccaccgtggccttagacctgccgcgggacgtggacgcgtcgatatcgttcgtgttctcgactcctccgtcgtcgtccgccgcgtaccgggcccagttgttcgtgaacggataccagtacggtcggtatcatccgcacatcggcaaccaggtcgtgtacccggttccaccgggcatcttggattaccagggcgacaacaccatcggggtcgcagtgtgggcgcagacggaggaaggggcacgggtggggttggactggcgcgtgaactatgtggcggatagttccttggatgtttctttcgacggggctgcgttgagaccggggtgggacgaggggcggttgcagtatgcatag

SEQ ID NO: 42 - protein, 1008 aa, Hamigera paravellanea
MTRLSEWAFVLLSTLGVFAAAQAQTVSQWPIHDNDLNTVVQWDHYSFIINGQRIFVFSGEFHYWRIPVPGLWRDILEKVKAAGFTAFAFYSSWAYHAPNNHTVDFSTGARDITPIFDLAKELGLYVIVRPGPYVNAEANAGGYPLWLTTGAYGSLRNNDTRYINALEPYFSKVSQITSQYQITNDHNTICYQIENEYGQQWIGSAYDRVPNETAIAYMEILKASARRNGIDIPLTANDPNMNTRSWGKDWSDEGGNVDIPGVDSYPSCWSCDLSVCTSTNGVYVPFQVLNYYDYFAETSPTMPSFMPEFQGGSYNPWGGPEGGCPDDIGPEFANLFYRWNIGQRVTAMSLYMLYGGTNWGAMAAPVTASSYDYSAPISEDRSIGAKYYETKLLGLFSRSARDLTVTDLIGNGTQYTNNVMIQARELRNPETNAAFYVTVHTNTSVSTNEVFHLRVNTSAGALTIPKHALGIRLNGHQSKIIVTDFTFGPRTLLYSTAEVLAYAALDDTPTLALWVPPGESGEFNVKGAKSGSVKKCQGCSNVQFHQENGGLTVAFTQSQGMSVVELNDGSRVVLLDRESAYRFWAPALTNDPFVPEDETVLIQGPYLVRGAKLSGSTLSVTGDIVNATTVEIFAPKTVKSITWNGRELKTSKTSYGSLQGSLKAPAPVKLPALTGWKSKDSLPERLASYDDSGAAWVDANHMTTLNPSPPATLPVLYADEYGFHNGVRLWRGYFNGTATGVFLNIQGGSAFGWSAYLNGHFLGSHLGAASIAQANRTLSFANATLNAFGPNVLLVIHDDTGHDQTTGALNPRGILNATLLSGDDSAQFTHWRLAGTAGGESNLDPVRGVYNEDGLFAERVGWHLPGFDDSAWPDASSPREGFAGATVRFYRTTVALDLPRDVDASISFVFSTPPSSSAAYRAQLFVNGYQYGRYHPHIGNQVVYPVPPGILDYQGDNTIGVAVWAQTEEGARVGLDWRVNYVADSSLDVSFDGAALRPGWDEGRLQYA

SEQ ID NO: 43 - protein, 985 aa, Hamigera paravellanea
  mat_peptide (1)..(985)
QTVSQWPIHDNDLNTVVQWDHYSFIINGQRIFVFSGEFHYWRIPVPGLWRDILEKVKAAGFTAFAFYSSWAYHAPNNHTVDFSTGARDITPIFDLAKELGLYVIVRPGPYVNAEANAGGYPLWLTTGAYGSLRNNDTRYINALEPYFSKVSQITSQYQITNDHNTICYQIENEYGQQWIGSAYDRVPNETAIAYMEILKASARRNGIDIPLTANDPNMNTRSWGKDWSDEGGNVDIPGVDSYPSCWSCDLSVCTSTNGVYVPFQVLNYYDYFAETSPTMPSFMPEFQGGSYNPWGGPEGGCPDDIGPEFANLFYRWNIGQRVTAMSLYMLYGGTNWGAMAAPVTASSYDYSAPISEDRSIGAKYYETKLLGLFSRSARDLTVTDLIGNGTQYTNNVMIQARELRNPETNAAFYVTVHTNTSVSTNEVFHLRVNTSAGALTIPKHALGIRLNGHQSKIIVTDFTFGPRTLLYSTAEVLAYAALDDTPTLALWVPPGESGEFNVKGAKSGSVKKCQGCSNVQFHQENGGLTVAFTQSQGMSVVELNDGSRVVLLDRESAYRFWAPALTNDPFVPEDETVLIQGPYLVRGAKLSGSTLSVTGDIVNATTVEIFAPKTVKSITWNGRELKTSKTSYGSLQGSLKAPAPVKLPALTGWKSKDSLPERLASYDDSGAAWVDANHMTTLNPSPPATLPVLYADEYGFHNGVRLWRGYFNGTATGVFLNIQGGSAFGWSAYLNGHFLGSHLGAASIAQANRTLSFANATLNAFGPNVLLVIHDDTGHDQTTGALNPRGILNATLLSGDDSAQFTHWRLAGTAGGESNLDPVRGVYNEDGLFAERVGWHLPGFDDSAWPDASSPREGFAGATVRFYRTTVALDLPRDVDASISFVFSTPPSSSAAYRAQLFVNGYQYGRYHPHIGNQVVYPVPPGILDYQGDNTIGVAVWAQTEEGARVGLDWRVNYVADSSLDVSFDGAALRPGWDEGRLQYA

SEQ ID NO: 44 - DNA, 3391 bp, Aspergillus unguis
  CDS (1)..(801)
  sig_peptide (1)..(60)
  mat_peptide (61)..(3388)
  CDS (847)..(1831)
  CDS (1883)..(2176)
  CDS (2236)..(2307)
  CDS (2368)..(2458)
  CDS (2527)..(3388)
atggcgcgagtctttcaactgcttctcttcctcctgggaagctttcagcttctgacagcagctcagaacagctcccaaaccgaatggcctgtacatgacaacgggctaagcgaggtcgtccaatgggaccattacagcttttacgttcacggccagcggttcttcctgttctcaggggaatttcactactggcgaatcccagtcccggccttgtggcgcgacattttggagaaggtcaaggcgcttgggttcaccggctttgcgttctactcaagctgggcataccatgcgcccaacaaccacacggtcgacttctcgaccggtgcgcgcaacatcaagcacatctttgaccttgcagaggagcttggaatgtacattattgtgcgacccggaccgtacgtcaacgctgaagcctctgctggtgggtttccgctctggcttacaacaggcgcgtatgggtcgacaaggaacgacgatcctagatataccgcggcgtggaagccatatttttctaaggtgtctgagatcacgagcaggtatcaggtcacggatggtcacaatacgttgatttaccagatcgagaatgagtatgggcagcagtggatcggggatccggtcgatagggaccttaacgagacagctgctgcttatatggatttgttgaaagcgacagctcgtgaaaacggaatcaaggtgcccttgactgcgaacgatcctaacatgggatcaaaatcttggggcaacgactggtcggatgctgcagggaacgtcgatgctgtggggttggactcttatccttctgtgagtgctcagtctccataatcaagtcctgtctaatcgatcaagtgctggagctgcgacgtcagcgtctgcacaggaacgaacggagaatacgtaccataccaagtaataaactactacgactacttcaacgaagtccagccaagcatgcctttcttcatgcccgaattccaaggaggatcgtataatccatggggtggccctgagggtggctgtcccgaggacaccggagcggactttgccaacttgttctacaggtggaatatcgggcagcgcgagacagccataagtctgtacatgattttcgggggaacaaactggggtggtatcgccgcgccagtcaccgcaaccagttatgactactccgctcctatctcagaggatcgatcgataggctcaaagttctacgagacaaagctgctagccctgttcacacgagctgcgaaagatttgactgtgactgatcgtgtcggcaacggaacgcagtatacgagcaataaagccgtcagcgcaattgagctgcgcaaccctgagaccaatacgggtttttacgtgaccagccacttggacactacaaccggcacagacgaggccttcaagctgcacgtcaacacctccgaaggggcattcaccatcccaaggctaaatggcaccataaggcttaatggccatcaatcaaagattatcgtcaccgacttcaaattcggcttcaagacgcttttatactcaaccgcagaggttctcacctacgcagtctttgaccataaaccaactctcgtcctttgggttcccactggtgaatcaggcgaattcgcaatcaaaggcgcgaaatcaggttctgcttcgactgcgtcggtgcagttccatcggcacggaagaacactgactgttgggtttacccaggctaaaggcctgagtgttctggagcttgataatggcgtcagagtagttttgctggatagggaggcggcgtatacgttctgggcacctgccttgacggacaatccgcttgttcctgagggtgaaagtggtgagttcccttttttctctctcttaataatcggtgatgctaataaagtagtccttgtcagcggaccctacctcgtccgatcctccaaactatccggatcaaccctagctctacgaggtgactcgctgggcgaaacaacactagaagtctttgctccaaacaatgtaaagaaggtgacatggaacggaaagaaggtcaaggtgtctaggaccaaatacgggagcctgaaagccaacctcgccgaaccgcgctctgtggaactgcccgctctcgacggatggaaggtcagcgacagcctgccagagaggttctcagactatgatgactcgggcaaggcttgggttggtatgttacatactccgtatacctggatctttgaagagataaaatactgacatgagcagccgcaaaccatctgacaacacccaatcccaataaaccagcgactctccccgttctctacgccaatgaatatggtattccgcctgaactctaactcggatcaaccagatcatgagctaacaacttgattccaggcttccacaacggcgtccgcctctggcgcggctactttaactcctctactgcgacgggcgtcttcctaaacatccaaggcggcgctgcattgtacgtccaaccaaacccctgccttctgtaaagccagtcatgaacagacataatactaataaacccagcggttggtccgcctggcttaacggccagctcattggctcgcacctaggcaacgcgacgatcgaacaagccaacgcaacactcccattcccggacaacaccctctccaagaacggagaacagaatgtgctcctcgtcgtccacgatgacacgggacatgaccagacaacgggtgtgctcaacccacgaggaatcctcgaagcgcgtctcctctcagacagtgaagaagagaatgaagacgagcaaggaggattcacgcattggcgcgtcgcgggagctgcaggcggcgaatcgaacctcgatcccgtccgaggtgtgtataacgaggatggactctacgcggagcgtgtgggttggcatttacctgggttcgacgacagcgagtggtctctcgcagacaatgcgaaggcaccactagccttcaccggcgcaacagtcaagttcttccggactgtcatacccccgttatcgatcccagagggcctcgacgtctccatctcgtttgtgttttccacggcgaatgtgtcgtccatctcgaccaccaccaccacaaactcaacggttggagaagaaaacaaaggcgataaatcggccttccgcgctcaactcttcgtcaacggctaccagtacggacggtacaatccaattgtcgggaaccaagttgcgtatcctgtcccgccggggattttggactacaatgacgagaatacggttggggttgcagtttgggcacagacggaggccggagcggaattcgggctcgattggaaagtcgattatgtgcttgagagttcgctggatgttgtgaatttggatgtggaggggttgaggccgaggtggagtgaggagagggagagatttgcgtag

SEQ ID NO: 45 - protein, 1035 aa, Aspergillus unguis
MARVFQLLLFLLGSFQLLTAAQNSSQTEWPVHDNGLSEVVQWDHYSFYVHGQRFFLFSGEFHYWRIPVPALWRDILEKVKALGFTGFAFYSSWAYHAPNNHTVDFSTGARNIKHIFDLAEELGMYIIVRPGPYVNAEASAGGFPLWLTTGAYGSTRNDDPRYTAAWKPYFSKVSEITSRYQVTDGHNTLIYQIENEYGQQWIGDPVDRDLNETAAAYMDLLKATARENGIKVPLTANDPNMGSKSWGNDWSDAAGNVDAVGLDSYPSCWSCDVSVCTGTNGEYVPYQVINYYDYFNEVQPSMPFFMPEFQGGSYNPWGGPEGGCPEDTGADFANLFYRWNIGQRETAISLYMIFGGTNWGGIAAPVTATSYDYSAPISEDRSIGSKFYETKLLALFTRAAKDLTVTDRVGNGTQYTSNKAVSAIELRNPETNTGFYVTSHLDTTTGTDEAFKLHVNTSEGAFTIPRLNGTIRLNGHQSKIIVTDFKFGFKTLLYSTAEVLTYAVFDHKPTLVLWVPTGESGEFAIKGAKSGSASTASVQFHRHGRTLTVGFTQAKGLSVLELDNGVRVVLLDREAAYTFWAPALTDNPLVPEGESVLVSGPYLVRSSKLSGSTLALRGDSLGETTLEVFAPNNVKKVTWNGKKVKVSRTKYGSLKANLAEPRSVELPALDGWKVSDSLPERFSDYDDSGKAWVAANHLTTPNPNKPATLPVLYANEYGFHNGVRLWRGYFNSSTATGVFLNIQGGAAFGWSAWLNGQLIGSHLGNATIEQANATLPFPDNTLSKNGEQNVLLVVHDDTGHDQTTGVLNPRGILEARLLSDSEEENEDEQGGFTHWRVAGAAGGESNLDPVRGVYNEDGLYAERVGWHLPGFDDSEWSLADNAKAPLAFTGATVKFFRTVIPPLSIPEGLDVSISFVFSTANVSSISTTTTTNSTVGEENKGDKSAFRAQLFVNGYQYGRYNPIVGNQVAYPVPPGILDYNDENTVGVAVWAQTEAGAEFGLDWKVDYVLESSLDVVNLDVEGLRPRWSEERERFA

SEQ ID NO: 46 - protein, 1015 aa, Aspergillus unguis
  mat_peptide (1)..(1015)
AQNSSQTEWPVHDNGLSEVVQWDHYSFYVHGQRFFLFSGEFHYWRIPVPALWRDILEKVKALGFTGFAFYSSWAYHAPNNHTVDFSTGARNIKHIFDLAEELGMYIIVRPGPYVNAEASAGGFPLWLTTGAYGSTRNDDPRYTAAWKPYFSKVSEITSRYQVTDGHNTLIYQIENEYGQQWIGDPVDRDLNETAAAYMDLLKATARENGIKVPLTANDPNMGSKSWGNDWSDAAGNVDAVGLDSYPSCWSCDVSVCTGTNGEYVPYQVINYYDYFNEVQPSMPFFMPEFQGGSYNPWGGPEGGCPEDTGADFANLFYRWNIGQRETAISLYMIFGGTNWGGIAAPVTATSYDYSAPISEDRSIGSKFYETKLLALFTRAAKDLTVTDRVGNGTQYTSNKAVSAIELRNPETNTGFYVTSHLDTTTGTDEAFKLHVNTSEGAFTIPRLNGTIRLNGHQSKIIVTDFKFGFKTLLYSTAEVLTYAVFDHKPTLVLWVPTGESGEFAIKGAKSGSASTASVQFHRHGRTLTVGFTQAKGLSVLELDNGVRVVLLDREAAYTFWAPALTDNPLVPEGESVLVSGPYLVRSSKLSGSTLALRGDSLGETTLEVFAPNNVKKVTWNGKKVKVSRTKYGSLKANLAEPRSVELPALDGWKVSDSLPERFSDYDDSGKAWVAANHLTTPNPNKPATLPVLYANEYGFHNGVRLWRGYFNSSTATGVFLNIQGGAAFGWSAWLNGQLIGSHLGNATIEQANATLPFPDNTLSKNGEQNVLLVVHDDTGHDQTTGVLNPRGILEARLLSDSEEENEDEQGGFTHWRVAGAAGGESNLDPVRGVYNEDGLYAERVGWHLPGFDDSEWSLADNAKAPLAFTGATVKFFRTVIPPLSIPEGLDVSISFVFSTANVSSISTTTTTNSTVGEENKGDKSAFRAQLFVNGYQYGRYNPIVGNQVAYPVPPGILDYNDENTVGVAVWAQTEAGAEFGLDWKVDYVLESSLDVVNLDVEGLRPRWSEERERFA

SEQ ID NO: 47 - DNA, 3859 bp, Aspergillus tamarii
  CDS (1)..(125)
  sig_peptide (1)..(66)
  mat_peptide (67)..(3856)
  CDS (189)..(243)
  CDS (299)..(321)
  CDS (371)..(415)
  CDS (477)..(948)
  CDS (1005)..(1139)
  CDS (1191)..(1210)
  CDS (1269)..(1289)
  CDS (1342)..(1544)
  CDS (1594)..(1686)
  CDS (1743)..(1780)
  CDS (1835)..(1985)
  CDS (2051)..(2464)
  CDS (2523)..(2816)
  CDS (2886)..(3856)
atgctcatctccaagaccgtgttcagcgggcttgccttgggggcgtcctttgttggcgtttctggtcagcagaattcaagccgttggccgttgcacgacaacggtttgacagacactgtagaatggtgggttcagtcaaattgcgaattcaaggctgtttggttggctctgacaccatggctatacagggatcactatagtttcttgattaatggtcagagacatttcgttttctctggagaggtttgtccgcccaatcccctatattctgtatattcaatacattaacatcatatagttccattactggcgtatccctgtgtaaggcaagagtcccacaacggcaacgctctagctaatggattaccagacccgaattatggagagatctactcgagaagatcaaagccgctgggtaggtagtctcagattcttgacgcccgttgtcaacaacacgctaataacgaattggatagtttcactgccttttccatctacaatcactggggatatcatacccccaagcccggcgttctcgacttcgagaacggggcccacaacttcacttcgatcatgactctagccaaagagataggtctctacatgattatccgaccgggcccatacgtcaatgcggaagccaatgctggcggtctccctctgtgggcaactacaggtgcctacggaaaactacgggataacgaccctcggtacttggaggctttgaccccatactgggctaacatttctaaaatcattgctcctcatctcatcaccaacggcggaaatgtcatcctgtatcagatcgagaatgagtacgccgagcagtggcttgacgaggaaacccaggagcccaacacgtctggtcaggaatacatgcagtatttggaggacgttgctcgggaaaacggcattgatgctcctctgatccataatcttccgaacatggtagggcaatacgctcgcttgctgaagatacagaatttttggctgatacatagcagaacggtcactcatggtccaaggacctctccaacgctactggaaatgtcgatgtcattggcgtggacagctatcccacttgctggacctgcaatgtcagtgagtgtctctcaactaacggagagtatatcccatatgtaagtaacgcctgcctttctttggtgatttattatactaaactctctcagaaaaccttgacctactacgagtaagtgcaatagtacacggatttgtatgagtgaaacactaatttaccctcaaatcagctacttcaagaaactatcaccgtaagctttgccctctctgagactatctacacattctaattctctattacagcactcagccaagctttatgcccgagttccaaggcggttcatacaacccatggggtggaccccaaggaggctgcccggatgatcttggcccggatttcgcgaacctcttctaccgaaacctaatctatcagagagtcagtgctatctcgctgtacatgttatacggcggtacaaactggggctggcacggctcaacagatgtcggtgagttattcccaagtcgaatttatgccacaggtgctgatgagcccagcgacaagttacgattactcttctccaatttcggagaaccgaaagcttattgagaaatactacgagacaaaagtgctcactcaattcacgaaaagtacgcctcttttagtacgatatgtggaagcttgccaagctaacctcatgatacagtcgcccgggatctgtctaaagtcgatcgtttaggcaacgtaagtagagcagaacaatatcgtctacagagaaacgctaacaggggtcaacagagcacgagatattcaagtaacccagctgtttcagtttctgagctgcgaaatcctgacaatggcgcggctttctacgtaactcagcacgaatacactccatctggaacggtcgaaaagttcacagtcaaggttaacacatccgatggtgctcgtatgttacctcctgcggtctgaatttggtatatcacaatgataatctgctaattactcgacaagtcactattcctcaatacggctcccaaatcactctcaatggtcaccagtccaagattatcgtcacagacttcaacttcggctcgaagacgctcctttactctacggcagaagttcttacctatgctgttattgatggtaaagaagtgctggctctctgggtcccgactggtgaatctggagagttcaccgtgaagggagtgaattcggccaagttcgccgacaaaggacgcactgcgaacatcgagattcgccccggagcaaacaaggtgacagtatctttcatgcagagagcgggtatgagcgtggttgagcttggtgatggaacacgcattgttcttctcgatcggtctgctgctcatgtattctggtctcctccactcaacaatgaccctgccgaggccggcaacaacactggtaagtccacatcgatggcgttatacaaacagttgatagactcgctgacatgcttcagtcctcgtccatggtccctacttagttcgctcggctagattggaaggctgtgacttgaagctcactggagatatccagaattctacaaaggtcagcatctttgcgcccaattcggtatgctccgtcaattggaatggcaagaagacatccgtcaagtcagcgaagggtggtgtcataaccacaaccttgggaggcgatgccaagttcgaacttcccacgatctccggctggaagtatgcggacagtctccctgaaatcgcgaaggactattccgctacaagcaaggcttgggttggtatgttatttctctcctcctcggtcgccaatagcacccgccagtgccagctaacaacagaaaaaccagtggctacgaagacaaactcgtctaatccgactcccccggcaccaaacaacccagtcctctacgtggacgagaacgatatccacgtcggcaaccacatctaccgcgccactttccccagcaccgacgagcccccaaccgacgtctacctcaacatcaccggaggtcgcgcattcggctactctgtctggctgaactcagaattcatcggctcctggctcggcaccccgacaaccgagcagaacgaccagacattctcattctccaacgcaaccctcagcacagacggagacaacatcctagtcgtcgtcatggacaactcggcccacgatctgcgcgagggagcaaccgacccccgaggaatcacaaacgccactctcgtcggtcccggaacctactccttcaccgagtggaaactcgccggcaacgcaggcttcgaagaccaccttgatccggtccgcgccccgctcaacgagggcagtctgtacgccgagcgagtcggtatccatctcccgggatatcagttcgacgaggccgaagaggtgccttcgaacagcacgagcctaaccgttcccggtgctggtattcgcgtcttccgcaccgttgttcccctctccgtgccccagggactggacgtctctatctcgttccgtttgactgctccctcgaatgtgacctttacctctacggagggatacaccaaccagctgcgcgctctgctcttcgttaatggataccagtatggtcgctttaacccttacatcggtcatcagattgacttccctgttcctccgggcgtccttgattataatggggataacacgattgcggtgacggtgtggagtcagagtgtggatggtgctgagatgaaaattgattggaatgtggactatgtccatgagaccagcttcgacatgaactttgacggagcatacctgagacctggatggatcgaggagagacgtgaatatgcttaa

SEQ ID NO: 48 - protein, 1020 aa, Aspergillus tamarii
MLISKTVFSGLALGASFVGVSGQQNSSRWPLHDNGLTDTVEWDHYSFLINGQRHFVFSGEFHYWRIPVPELWRDLLEKIKAAGFTAFSIYNHWGYHTPKPGVLDFENGAHNFTSIMTLAKEIGLYMIIRPGPYVNAEANAGGLPLWATTGAYGKLRDNDPRYLEALTPYWANISKIIAPHLITNGGNVILYQIENEYAEQWLDEETQEPNTSGQEYMQYLEDVARENGIDAPLIHNLPNMNGHSWSKDLSNATGNVDVIGVDSYPTCWTCNVSECLSTNGEYIPYKTLTYYDYFKKLSPTQPSFMPEFQGGSYNPWGGPQGGCPDDLGPDFANLFYRNLIYQRVSAISLYMLYGGTNWGWHGSTDVATSYDYSSPISENRKLIEKYYETKVLTQFTKIARDLSKVDRLGNSTRYSSNPAVSVSELRNPDNGAAFYVTQHEYTPSGTVEKFTVKVNTSDGALTIPQYGSQITLNGHQSKIIVTDFNFGSKTLLYSTAEVLTYAVIDGKEVLALWVPTGESGEFTVKGVNSAKFADKGRTANIEIRPGANKVTVSFMQRAGMSVVELGDGTRIVLLDRSAAHVFWSPPLNNDPAEAGNNTVLVHGPYLVRSARLEGCDLKLTGDIQNSTKVSIFAPNSVCSVNWNGKKTSVKSAKGGVITTTLGGDAKFELPTISGWKYADSLPEIAKDYSATSKAWVVATKTNSSNPTPPAPNNPVLYVDENDIHVGNHIYRATFPSTDEPPTDVYLNITGGRAFGYSVWLNSEFIGSWLGTPTTEQNDQTFSFSNATLSTDGDNILVVVMDNSAHDLREGATDPRGITNATLVGPGTYSFTEWKLAGNAGFEDHLDPVRAPLNEGSLYAERVGIHLPGYQFDEAEEVPSNSTSLTVPGAGIRVFRTVVPLSVPQGLDVSISFRLTAPSNVTFTSTEGYTNQLRALLFVNGYQYGRFNPYIGHQIDFPVPPGVLDYNGDNTIAVTVWSQSVDGAEMKIDWNVDYVHETSFDMNFDGAYLRPGWIEERREYA

SEQ ID NO: 49 - protein, 998 aa, Aspergillus tamarii
  mat_peptide (1)..(998)
QQNSSRWPLHDNGLTDTVEWDHYSFLINGQRHFVFSGEFHYWRIPVPELWRDLLEKIKAAGFTAFSIYNHWGYHTPKPGVLDFENGAHNFTSIMTLAKEIGLYMIIRPGPYVNAEANAGGLPLWATTGAYGKLRDNDPRYLEALTPYWANISKIIAPHLITNGGNVILYQIENEYAEQWLDEETQEPNTSGQEYMQYLEDVARENGIDAPLIHNLPNMNGHSWSKDLSNATGNVDVIGVDSYPTCWTCNVSECLSTNGEYIPYKTLTYYDYFKKLSPTQPSFMPEFQGGSYNPWGGPQGGCPDDLGPDFANLFYRNLIYQRVSAISLYMLYGGTNWGWHGSTDVATSYDYSSPISENRKLIEKYYETKVLTQFTKIARDLSKVDRLGNSTRYSSNPAVSVSELRNPDNGAAFYVTQHEYTPSGTVEKFTVKVNTSDGALTIPQYGSQITLNGHQSKIIVTDFNFGSKTLLYSTAEVLTYAVIDGKEVLALWVPTGESGEFTVKGVNSAKFADKGRTANIEIRPGANKVTVSFMQRAGMSVVELGDGTRIVLLDRSAAHVFWSPPLNNDPAEAGNNTVLVHGPYLVRSARLEGCDLKLTGDIQNSTKVSIFAPNSVCSVNWNGKKTSVKSAKGGVITTTLGGDAKFELPTISGWKYADSLPEIAKDYSATSKAWVVATKTNSSNPTPPAPNNPVLYVDENDIHVGNHIYRATFPSTDEPPTDVYLNITGGRAFGYSVWLNSEFIGSWLGTPTTEQNDQTFSFSNATLSTDGDNILVVVMDNSAHDLREGATDPRGITNATLVGPGTYSFTEWKLAGNAGFEDHLDPVRAPLNEGSLYAERVGIHLPGYQFDEAEEVPSNSTSLTVPGAGIRVFRTVVPLSVPQGLDVSISFRLTAPSNVTFTSTEGYTNQLRALLFVNGYQYGRFNPYIGHQIDFPVPPGVLDYNGDNTIAVTVWSQSVDGAEMKIDWNVDYVHETSFDMNFDGAYLRPGWIEERREYA

SEQ ID NO: 50 - DNA, 3197 bp, Curvularia spicifera
  CDS (1)..(265)
  sig_peptide (1)..(81)
  mat_peptide (82)..(3194)
  CDS (320)..(917)
  CDS (973)..(1925)
  CDS (1981)..(3194)
atgaagactttcgttgggctctcgtggctgtcggccttgtcttcgttggtgacgctcccaaatggctccggtgttgctgcccagaacaacacgcctagtacgtggccgctccacgacaatggtctgaatgatgtcgtacaatgggatcattattcctttaaagtgaacggaaagcgccttttcgttttctctggagaaattcactactggcgtatcccggtctatgaggtttgggaggacttgttagaaaaaattaaggcggctggtaagtatttccatttgcataagatgcatgtcgattacggctgacgaccattaggtttcacggctttcgccttctacggcaactgggcctatcacagcgcaaacaaccagaccttggactttgaaagcggcgcgcacgactttacgaagctcttcgagatcgcggagcgcgtcggcctttacgtcattaccaggcctggtccttatgtcaatgctgaggcgaacgctggaggcttcccattatggctcactacgggagcttatggaacgctacgcaacgacgaccccagatacctccaagcattggacccttacttctccaagttctctgagctcacatccaagcatctcgtgaccaagggcggaaaagcgcttgtctaccagatcgagaacgagtatggtgagcagtggaagaatagagaccagaagattcccaatgaaagtgccggaagatatatgcaggcgcttgaggatttggcacgggctcatggcattgacgtccccctaatccacaacgaccccaatatgaacaccaagagctggagcaaagactatgcccctggtgctgtaggaaatgtcgatgttgctgggctcgacagctacccatcctgttggtcctgcaacctggatgagtgcacgggtaccaatggagagtaagtgttgtaaatctcaaacgctccagtaacagttactaacgttatgttctagatacgtagcataccaaaccatcaactactttgatcatttcgaagaagtatctccaacccagccaagcttcttccctgaattccaaggtggttcgtacaatccttggggtggacccgaaggtggctgtcccggtgacattggagctgatttcgcaaatctcttctaccgaaacctggtctcccaacgcgttaccgcaatctcactttatatggtttttggcggcacaaattggggcgccattgcagccccagtcacagccacgtcgtatgactatagcagtcctatcagcgagaaccgggagattggcgccaaattctacgagacgaagaacttggctttgttcactcgtgttgcggaagacttgacagttaccgatcgccttggaaattctacttcttacacgaccaactcggcagtcgaggcgagtgaactccgcaacccacacaccaacggcgcattttacgttaccattcatgccacatcgtcttccgcgacgaaggaatcattcaagctccatgtgagcacatccatcggtaatctcactatccctcaacatgctggttctattgttctcgatggccatcaatccaagatccttgttaccgatttcgcaatgggcaacagtaccttgacatactccactgcagaagttgtcacctacgctcttatcgactccaagccagttgttttgctatcaactggtattggcgagtctgctgaattccatgtcaagggcgctaagaagggttccgctgtcagcagtggtgctagctcgaatgctacgttctacaccgaggccggtggtgttacgaccagcatacagaaagtttcgggtatgagcgtctaccagttcgataatggtgtgaaggttgttgttgcggataagcctaccgcgtacctgttctgggcacctaacctgtcgaacgacccctttgcgcccgttgatcaatccggtaagtatactaaattcgtgattcttctggttctcgaaatctaacatgcacatagttttggtccagggaccatacctcgtccgccacgtagctctcgacggccacgtcctcgccctgaaaggagatatcatgaacagcactgacatcgaagtctttgcctgtcacaatgccaaaactctgtcctggaatggaaagaagctctctacctcgcgaacctcgtacggtagtctgaaagcccacatcaccgctttcaacggcactattcagctaccttccctcgacaactggaaagtcaacgaaggtctcccagagaaggaggcagattacgatgacagcagcgccgcttgggttatagccgaccacctcagcacccccaaccctaccaagcccgacactcttcccgttctgtacgtcgatgagtatggcttccacaacagcttccaccttttccgcggctacttcgatggctccgccaccggcgtccaactctctgtgcaaggcggtctcgcatttggctggagtgcctggctaaacggcaaacatattggttcttggctgggcaatacgaccctcggtgtaggcaacgcaacgctctcctttgccaacgccacagttcactccaatggaaccaacgtcctcctcgtcgcccaagacaacacaggccacgatctccgcggcggcgccaccgatccccgcggtatcctgcgcgcatccctttccggcccctcaaacttcacaagctggaaaatcgcaggtgaagccggcggcgaatccatccagctcgaccccgtccgtggtcccctggctgaaggcggcctcgtcgctgaacgccttggctggcacctccctggcttcgacgacgcggactgggccaccagctcgccttccgccggattctcaggcgcagatataaagttctaccgtactacattcccgcttgatgtacctgaccatgttgatgcttccttcgcatttgtgctgaacgcccctgctgcgaagacgattcgcgtccagctttttgtcaatgggtatcagtatgcgcggtttaatccgtatgtgggtaatgaaatcaagttccctgttcctccgggcattctcaactacagcggagagaatgtggttgggctgagtgtgtgggcacaagaggaagacggagcaaaggtcgatgtgcgtatggtgcaggagtttgcggttgaaagtagttggaaatcgaggtttaatggcgagtatttgaggccgaagtggacagaggagagactggagtatgcttga

SEQ ID NO: 51 - protein, 1010 aa, Curvularia spicifera
MKTFVGLSWLSALSSLVTLPNGSGVAAQNNTPSTWPLHDNGLNDVVQWDHYSFKVNGKRLFVFSGEIHYWRIPVYEVWEDLLEKIKAAGFTAFAFYGNWAYHSANNQTLDFESGAHDFTKLFEIAERVGLYVITRPGPYVNAEANAGGFPLWLTTGAYGTLRNDDPRYLQALDPYFSKFSELTSKHLVTKGGKALVYQIENEYGEQWKNRDQKIPNESAGRYMQALEDLARAHGIDVPLIHNDPNMNTKSWSKDYAPGAVGNVDVAGLDSYPSCWSCNLDECTGTNGEYVAYQTINYFDHFEEVSPTQPSFFPEFQGGSYNPWGGPEGGCPGDIGADFANLFYRNLVSQRVTAISLYMVFGGTNWGAIAAPVTATSYDYSSPISENREIGAKFYETKNLALFTRVAEDLTVTDRLGNSTSYTTNSAVEASELRNPHTNGAFYVTIHATSSSATKESFKLHVSTSIGNLTIPQHAGSIVLDGHQSKILVTDFAMGNSTLTYSTAEVVTYALIDSKPVVLLSTGIGESAEFHVKGAKKGSAVSSGASSNATFYTEAGGVTTSIQKVSGMSVYQFDNGVKVVVADKPTAYLFWAPNLSNDPFAPVDQSVLVQGPYLVRHVALDGHVLALKGDIMNSTDIEVFACHNAKTLSWNGKKLSTSRTSYGSLKAHITAFNGTIQLPSLDNWKVNEGLPEKEADYDDSSAAWVIADHLSTPNPTKPDTLPVLYVDEYGFHNSFHLFRGYFDGSATGVQLSVQGGLAFGWSAWLNGKHIGSWLGNTTLGVGNATLSFANATVHSNGTNVLLVAQDNTGHDLRGGATDPRGILRASLSGPSNFTSWKIAGEAGGESIQLDPVRGPLAEGGLVAERLGWHLPGFDDADWATSSPSAGFSGADIKFYRTTFPLDVPDHVDASFAFVLNAPAAKTIRVQLFVNGYQYARFNPYVGNEIKFPVPPGILNYSGENVVGLSVWAQEEDGAKVDVRMVQEFAVESSWKSRFNGEYLRPKWTEERLEYA

SEQ ID NO: 52 - protein, 983 aa, Curvularia spicifera
  mat_peptide (1)..(983)
QNNTPSTWPLHDNGLNDVVQWDHYSFKVNGKRLFVFSGEIHYWRIPVYEVWEDLLEKIKAAGFTAFAFYGNWAYHSANNQTLDFESGAHDFTKLFEIAERVGLYVITRPGPYVNAEANAGGFPLWLTTGAYGTLRNDDPRYLQALDPYFSKFSELTSKHLVTKGGKALVYQIENEYGEQWKNRDQKIPNESAGRYMQALEDLARAHGIDVPLIHNDPNMNTKSWSKDYAPGAVGNVDVAGLDSYPSCWSCNLDECTGTNGEYVAYQTINYFDHFEEVSPTQPSFFPEFQGGSYNPWGGPEGGCPGDIGADFANLFYRNLVSQRVTAISLYMVFGGTNWGAIAAPVTATSYDYSSPISENREIGAKFYETKNLALFTRVAEDLTVTDRLGNSTSYTTNSAVEASELRNPHTNGAFYVTIHATSSSATKESFKLHVSTSIGNLTIPQHAGSIVLDGHQSKILVTDFAMGNSTLTYSTAEVVTYALIDSKPVVLLSTGIGESAEFHVKGAKKGSAVSSGASSNATFYTEAGGVTTSIQKVSGMSVYQFDNGVKVVVADKPTAYLFWAPNLSNDPFAPVDQSVLVQGPYLVRHVALDGHVLALKGDIMNSTDIEVFACHNAKTLSWNGKKLSTSRTSYGSLKAHITAFNGTIQLPSLDNWKVNEGLPEKEADYDDSSAAWVIADHLSTPNPTKPDTLPVLYVDEYGFHNSFHLFRGYFDGSATGVQLSVQGGLAFGWSAWLNGKHIGSWLGNTTLGVGNATLSFANATVHSNGTNVLLVAQDNTGHDLRGGATDPRGILRASLSGPSNFTSWKIAGEAGGESIQLDPVRGPLAEGGLVAERLGWHLPGFDDADWATSSPSAGFSGADIKFYRTTFPLDVPDHVDASFAFVLNAPAAKTIRVQLFVNGYQYARFNPYVGNEIKFPVPPGILNYSGENVVGLSVWAQEEDGAKVDVRMVQEFAVESSWKSRFNGEYLRPKWTEERLEYA

SEQ ID NO: 53 - DNA, 3829 bp, Aspergillus oryzae
  CDS (1)..(125)
  sig_peptide (1)..(66)
  mat_peptide (67)..(3826)
  CDS (195)..(249)
  CDS (306)..(328)
  CDS (378)..(422)
  CDS (481)..(952)
  CDS (1009)..(1143)
  CDS (1193)..(1212)
  CDS (1266)..(1286)
  CDS (1337)..(1539)
  CDS (1588)..(1680)
  CDS (1735)..(1772)
  CDS (1826)..(1976)
  CDS (2035)..(2448)
  CDS (2507)..(2800)
  CDS (2856)..(3826)
atgctcatctccaagaccgtgctcagcggacttgccttgggggcgtccttcgttggcgtttctgctcagcagaactcaacccgttggccgttgcatgacaacggcttgacagacactgtagaatggtaggtttagccaatttgtggattcatttgtggatcaatactgttagctctgacaccatggctatacagggatcactatagtttcttgattaatggtcagagacattttgttttctctggagaggttggtccacccaatcgtttatgttctacatggttcaatgcattaacatcgtatagttccattactggcgtattcctgtgtaaggcaagagtcctacaacggcagcgctctcgctaatatataaccaggcccgaattatggagagatctactggagaagatcaaggccgctgggtaggtagttccagattttgaaagtcgtttctcggcacgctaatggcaaattcgacagtttcactgccttttccatctacaatcactggggataccacagccctaaacccggtgttctcgactttgagaacggagcccacaatttcacctcgatcatgactctagccaaagagataggtctctacatgatcatccggccgggcccatacgtcaatgcagaagccaatgctggcggtctccctctgtggacgactacaggtgcctacgggaaactgcgggataacgaccctcggtatctggaggctttgaccccgtactgggctaacatttctaaaattattgcccctcatctcatcactaatgacggaaatgtaatcctgtatcagatcgaaaatgagtacgccgagcagtggcttgatgaggaaacccacgagcccaacacgtctggtcaggaatacatgcagtatttggaggatgttgctcgggaaaatggcattgatgctcctctgatccataatcttcccaacatggtagggcaatatgctcacttactgaagatacagaatatttggctgatgtataacagaacggtcactcatggtccaaggacctctccaacgccaccggaaatgtcgatgtcattggcgtggacagctatcccacttgctggacctgcaatgtcagtgagtgtgcttcaactaacggagagtatatcccatatgtaagtaggactttgtctttgtctggaggttcatgctaatttacctcagaaaaccttgatctactacgagtaagtgtgatgcacagactgtacgagttaaaactgacttaccctcaaattagctactttaaggaattatcaccgtgagtttgctctacttgagactacccacacattctaacgcctatcatagcactcaaccaagcttcatgcccgagttccaaggcggctcgtacaacccatggggtggacctcaaggcggctgcccggatgaccttggcccggattttgcgaatctcttctaccgaaacttgatctcccagagagtcagcgctatctcgttgtacatgttgtacggcggtaccaactggggctggcacgcctcaacggatgtcggtaagttatccccaatccaacttatgctataggtgttgatgagcccagcgacgagctacgactactcctccccaatttcggagaaccgaaagctcattgagaaatactatgagacgaaagtactcactcaattcacgaaaagtacgcctctttatccgataggtggaagctcgccaagctaatctcaggatacagtcgcccaggatctgtctaaggtcgaccggttaggcaacgtaagtagatgataacaatatcgtgtaccgagaaacattaaccaagttaatagagcacgaaatactcgagcaatccagcagtgtcggttgctgagctgcggaaccctgacactggcgcggctttctacgtaactcagcacgagtacactccatctggaacggttgaaaagttcacggtcaaggttaacacttccgagggtgctcgtatgttatctcctctagtacccatatcgcaatgatcaactgctgacttcttgacaagttactattcctcagtatggctcccaaatcactctcaacggtcaccaatccaagatcattgtcacggacttcaagttcggctcgaagacactcctttactctacggcggaggttcttacctacgctgttattgatggcaaagaagtgctggctctctgggtccctactggagaatcgggagaattcaccgtgaagggagtgaattcggctaagttcgccgacaaagggcgtactgcgaacatcgagattcaccctgggacaaacaatgtaacagtctctttcatgcagagatcgggtatgagcctggttgagcttggtgatggaacacgcattgttcttctcgatcggtctgctgctcatgtattctggtctactccactcaacaatgaccctgccgaggctggcaacaacactggtgagtccccatcgatggcggtatacaaacagttgataggctcgctgacactcctcagtccttgtccatggcccctacttagttcgctcggctaaactggaaggctgtgacttgaaactcactggagatatccagaactctacagaggtcagcatctttgcacccaagtctgtatgctctgtcaattggaatggcaagaagacatccgtcaagtcggcgaagggtggtgttataaccacaaccctgggaggcgatgccaagttcgagcttcccacgatctctggctggaagtctgcggacagtctccctgaaatcgcaaaggactactccgctacaagcaaggcttgggttggtatgttaccctctcctccacggccaatagtacccaccagctaacaaaagaccagtggctacaaagacaaactcgtctaaccctactcccccggcaccgaacaacccagtcctctacgtagacgagaacgatatccacgtcggcaaccacatctaccgcgccacattccccagcaccgacgagcctccaaccgacgtctacctcaacatcaccggaggtcgcgcattcggctactcagtctggctgaactccgacttcatcggctcctggctcggcactgcgacaactgagcaaaacgaccagacattctccttctccaacgcaaccctcagcacagacgaagacaacatcctagtcgtcgtcatggacaactcagcccacgacttgcgcgacggagcactcaacccccgaggcatcacaaacgccaccctcatcggtcccggaagctactccttcaccgagtggaaactggccggcaacgcaggcttcgaagaccaccttgacccggtccgcgccccgctcaacgagggcagtctgtacgccgagcgcgtcggtatccatctcccgggctatgagttcgacgaagccgaggaggtgtcttcaaacagcacgagcctaaccgttcccggcgctggtattcgcgtcttccgcactgttgttcccctctccgtgccccagggactggacgtctctatctcgttccgtctgacggcgccctcgaacgtaacctttacctctgcggaggggtatactaaccagctgcgggctctgcttttcgtcaatgggtaccagtatggtcgctttaacccctatatcggtcatcagatcgacttccctgttcctccgggtgtccttgattacaacggggataacacgattgccgtgacggtgtggagtcagagtgtggatggtgctgagatcaaggtcgattggaatgtggactatgtccatgagaccagcttcgatatgaactttgatggagcgtacctgagacctggatggatcgaggagagacgtgaatatgcttaa

SEQ ID NO: 54 - protein, 1020 aa, Aspergillus oryzae
MLISKTVLSGLALGASFVGVSAQQNSTRWPLHDNGLTDTVEWDHYSFLINGQRHFVFSGEFHYWRIPVPELWRDLLEKIKAAGFTAFSIYNHWGYHSPKPGVLDFENGAHNFTSIMTLAKEIGLYMIIRPGPYVNAEANAGGLPLWTTTGAYGKLRDNDPRYLEALTPYWANISKIIAPHLITNDGNVILYQIENEYAEQWLDEETHEPNTSGQEYMQYLEDVARENGIDAPLIHNLPNMNGHSWSKDLSNATGNVDVIGVDSYPTCWTCNVSECASTNGEYIPYKTLIYYDYFKELSPTQPSFMPEFQGGSYNPWGGPQGGCPDDLGPDFANLFYRNLISQRVSAISLYMLYGGTNWGWHASTDVATSYDYSSPISENRKLIEKYYETKVLTQFTKIAQDLSKVDRLGNSTKYSSNPAVSVAELRNPDTGAAFYVTQHEYTPSGTVEKFTVKVNTSEGALTIPQYGSQITLNGHQSKIIVTDFKFGSKTLLYSTAEVLTYAVIDGKEVLALWVPTGESGEFTVKGVNSAKFADKGRTANIEIHPGTNNVTVSFMQRSGMSLVELGDGTRIVLLDRSAAHVFWSTPLNNDPAEAGNNTVLVHGPYLVRSAKLEGCDLKLTGDIQNSTEVSIFAPKSVCSVNWNGKKTSVKSAKGGVITTTLGGDAKFELPTISGWKSADSLPEIAKDYSATSKAWVVATKTNSSNPTPPAPNNPVLYVDENDIHVGNHIYRATFPSTDEPPTDVYLNITGGRAFGYSVWLNSDFIGSWLGTATTEQNDQTFSFSNATLSTDEDNILVVVMDNSAHDLRDGALNPRGITNATLIGPGSYSFTEWKLAGNAGFEDHLDPVRAPLNEGSLYAERVGIHLPGYEFDEAEEVSSNSTSLTVPGAGIRVFRTVVPLSVPQGLDVSISFRLTAPSNVTFTSAEGYTNQLRALLFVNGYQYGRFNPYIGHQIDFPVPPGVLDYNGDNTIAVTVWSQSVDGAEIKVDWNVDYVHETSFDMNFDGAYLRPGWIEERREYA

SEQ ID NO: 55 - protein, 998 aa, Aspergillus oryzae
  mat_peptide (1)..(998)
QQNSTRWPLHDNGLTDTVEWDHYSFLINGQRHFVFSGEFHYWRIPVPELWRDLLEKIKAAGFTAFSIYNHWGYHSPKPGVLDFENGAHNFTSIMTLAKEIGLYMIIRPGPYVNAEANAGGLPLWTTTGAYGKLRDNDPRYLEALTPYWANISKIIAPHLITNDGNVILYQIENEYAEQWLDEETHEPNTSGQEYMQYLEDVARENGIDAPLIHNLPNMNGHSWSKDLSNATGNVDVIGVDSYPTCWTCNVSECASTNGEYIPYKTLIYYDYFKELSPTQPSFMPEFQGGSYNPWGGPQGGCPDDLGPDFANLFYRNLISQRVSAISLYMLYGGTNWGWHASTDVATSYDYSSPISENRKLIEKYYETKVLTQFTKIAQDLSKVDRLGNSTKYSSNPAVSVAELRNPDTGAAFYVTQHEYTPSGTVEKFTVKVNTSEGALTIPQYGSQITLNGHQSKIIVTDFKFGSKTLLYSTAEVLTYAVIDGKEVLALWVPTGESGEFTVKGVNSAKFADKGRTANIEIHPGTNNVTVSFMQRSGMSLVELGDGTRIVLLDRSAAHVFWSTPLNNDPAEAGNNTVLVHGPYLVRSAKLEGCDLKLTGDIQNSTEVSIFAPKSVCSVNWNGKKTSVKSAKGGVITTTLGGDAKFELPTISGWKSADSLPEIAKDYSATSKAWVVATKTNSSNPTPPAPNNPVLYVDENDIHVGNHIYRATFPSTDEPPTDVYLNITGGRAFGYSVWLNSDFIGSWLGTATTEQNDQTFSFSNATLSTDEDNILVVVMDNSAHDLRDGALNPRGITNATLIGPGSYSFTEWKLAGNAGFEDHLDPVRAPLNEGSLYAERVGIHLPGYEFDEAEEVSSNSTSLTVPGAGIRVFRTVVPLSVPQGLDVSISFRLTAPSNVTFTSAEGYTNQLRALLFVNGYQYGRFNPYIGHQIDFPVPPGVLDYNGDNTIAVTVWSQSVDGAEIKVDWNVDYVHETSFDMNFDGAYLRPGWIEERREYA

SEQ ID NO: 56 - DNA, 3355 bp, Aspergillus carneus
  CDS (1)..(801)
  sig_peptide (1)..(60)
  mat_peptide (61)..(3352)
  CDS (870)..(1866)
  CDS (1916)..(2215)
  CDS (2267)..(2338)
  CDS (2389)..(2476)
  CDS (2530)..(3352)
atggcgcgtctcccacagctcctcttcctactcctcgcgagtgtcgggctcctcagcgcagcccagaaccacaccgactccgaatggccactccacgataacggcctaaacaccgtcgttcaatgggatcactacagcttccaggtccacggccagcgcatcttcgtcttctccggcgaatttcactactggcgcatccccgtcccgggactctggcgcgacatcctggagaagatcaaggctgccggattcactgcattcgctttctactccagctgggcctaccatgcacccaacaatcacactgtggacttctcgaccggcgcccgcgacatcacccccatctacgagctcgcgaaagagctgggcatgtatatcatcgtccgaccgggcccctacgtcaatgcggaggccagcgccggcggctatcccctgtgggtgaccaccggtgcatacggcagtctgcggaacgacgacgcacggtacaccgaggcctggaagccgtactttgccaaaatgtcggaaatcacgagccagtaccaggtcaccgatggccacaatacgttctgctatcagattgagaacgagtacggccagcaatggattggagatcccgtcgatcgaaaccccaaccagacggccgttgcgtacatggaactcctcgaagagagtgcccgcgaaaatggcatcgtcgtgccattgactgcgaatgaccccaacatgaacaccaagtcctgggggaatgattggtctaatgcagggggcaatgtcgatgttgtcgggctggattcttacccttctgtaagctattctccctcctatacaacacccctatacaagatctcctgaccaacaaactaatgatacagtgctggacttgcgacgtcacccaatgcacctccaccaacggagaatacgtgccctacaaggtgatggggtactacgactacttccaggaggtgcagcccaccatgccgggcttcatgcctgagttccagggtgggagttacaacccctgggccggcccggagggtggatgtcccggagacacgggagtcgactttgcgaatctcttctaccggtggaacatcgcgcagcgggtgacggctatgagtctgtacatgctgtacgggggcacgaactggggcgccatcgccgcgccggtcacggctaccagctacgactactcctcgcccatctcggaagaccgctccatcggcagcaaatactacgagaccaagctcctggcgctcttcacccgcagtgccacggacctgaccatgaccgaccgcatcggaaacggcacgcagtacacgaacaacccggctgtcgccgcctacgaactgcgtaaccccgtcaccaacggggcgttttacgtgaccatccatgcagacagcaccgtcggctcggatgagtcgttccggttgaacgtcaacacctccgcaggtgcgttcacggtccccagcaagggcgcaatccgtctcaacggacaccaatcgaagattgtcgtcacggacttccgcttcgggccctctcactcgttgctgtattccaccgcggaggtcctcacccatgcggtgttcgacaagcaggccactatcgtcctttgggttcccaccggggagtcgggcgaattcgccgtcaagggcgcaaagtccggtaaggtagaaagctgtccacggtgctccaacgcgaccttcactcggaagaaagatgtgctcgttgtcaactttacgcagactggcgggatgagtgtgctccagctgaacaacggcgtgcgcgtcgttcttcttgatcgtcccgctgcatacaacttctgggctcctccggtgaccgacgatccttttgccccagagaccgatctgggtaagatggcttcgcccttctaaggtcacaattcgttaacagtaggcagttctcgtccaaggcccatacctcgtgcgttccgcgagtctgtccgggtcgaccctcgcgctgagaggcgactcgatcaaagagaccgcgttggagatcttcgcacccaagaaggtgaagacagtcacctggaatgggaagcgagtcaagacttccaagtcatcatacgggagtctcaccgcgtcgctcgcacctccaccggctgtgacgctcccggcattgacctcgacccgatggaagtcccaagacagtctgcccgaaaggcttccatcctacgacgactccggaccggcctgggttggtacgtatctcgctacattctctctatgtcccgtactaacaacctacgcagacgccgaccacatgactacacagaaccccaggaccccggagaccctccccgtgctctacgcagatgaatacggtactatcaccctcactcacattccctcaaacacctcactaacggtacaggcttccacaatggcatccgcctctggcgcgggtccttcaccgacgctgcctcgggcgtctacctcaacgtccaaggcggcgccgccttgtacgtacattccctcctcatccctcccagcaccaactaacatacattcccagtggctggtccgcctacctgaacggccacttcctcggctcccacctcggcacagcaacaacctcccaggcgaacaaaacgctcgtcttcccaaccggtgcactcaaccaaaacgccaccaacaccctcctcgtcatccatgacgacaccggccacgaccagaccaccggcgcgctgaacccgcgcggcatcctcgccgcccggctgctccccgcctccaacgccgcggccgactcgaccgccccgaccttcacacggtggcgcgtcgccggcacagcgggcggggaatccgacctcgaccccgtacgcggcgtctacaacgaagacgggctcttcgcggagcgcgtcggctggcacctccccggcttcgacgacggcgcctggcccgccgccaacacgaccgccgtggcgcaagaaaccggaaccgtgtcgctgtccttcaccggagcaacggtgcgcttcttccgcaccgtcatcccgctgcatctgccgcgcggcatcgacgcgtccatctcgttcgtgctgggcacgcctgccggcacgtccaccgcgtaccgcgcccagctgttcgtcaacggctaccagtacggccggtactacccgcacatcgggaaccaggtggtgtacccggttccggcgggagtgctggactacgacggtgagaacacgatcggcgtggcggtgtgggcgcagagtgacgccggggcggcgatcaatctggactggcgggtgaactacgttgccgacagctcgttggacgcggtgcggcttaccggggaggggtcgttaagaccccagtggagtgaggcaagagagcggtacgcttag

SEQ ID NO: 57 - protein, 1027 aa, Aspergillus carneus
MARLPQLLFLLLASVGLLSAAQNHTDSEWPLHDNGLNTVVQWDHYSFQVHGQRIFVFSGEFHYWRIPVPGLWRDILEKIKAAGFTAFAFYSSWAYHAPNNHTVDFSTGARDITPIYELAKELGMYIIVRPGPYVNAEASAGGYPLWVTTGAYGSLRNDDARYTEAWKPYFAKMSEITSQYQVTDGHNTFCYQIENEYGQQWIGDPVDRNPNQTAVAYMELLEESARENGIVVPLTANDPNMNTKSWGNDWSNAGGNVDVVGLDSYPSCWTCDVTQCTSTNGEYVPYKVMGYYDYFQEVQPTMPGFMPEFQGGSYNPWAGPEGGCPGDTGVDFANLFYRWNIAQRVTAMSLYMLYGGTNWGAIAAPVTATSYDYSSPISEDRSIGSKYYETKLLALFTRSATDLTMTDRIGNGTQYTNNPAVAAYELRNPVTNGAFYVTIHADSTVGSDESFRLNVNTSAGAFTVPSKGAIRLNGHQSKIVVTDFRFGPSHSLLYSTAEVLTHAVFDKQATIVLWVPTGESGEFAVKGAKSGKVESCPRCSNATFTRKKDVLVVNFTQTGGMSVLQLNNGVRVVLLDRPAAYNFWAPPVTDDPFAPETDLVLVQGPYLVRSASLSGSTLALRGDSIKETALEIFAPKKVKTVTWNGKRVKTSKSSYGSLTASLAPPPAVTLPALTSTRWKSQDSLPERLPSYDDSGPAWVDADHMTTQNPRTPETLPVLYADEYGFHNGIRLWRGSFTDAASGVYLNVQGGAAFGWSAYLNGHFLGSHLGTATTSQANKTLVFPTGALNQNATNTLLVIHDDTGHDQTTGALNPRGILAARLLPASNAAADSTAPTFTRWRVAGTAGGESDLDPVRGVYNEDGLFAERVGWHLPGFDDGAWPAANTTAVAQETGTVSLSFTGATVRFFRTVIPLHLPRGIDASISFVLGTPAGTSTAYRAQLFVNGYQYGRYYPHIGNQVVYPVPAGVLDYDGENTIGVAVWAQSDAGAAINLDWRVNYVADSSLDAVRLTGEGSLRPQWSEARERYA

SEQ ID NO: 58 - protein, 1007 aa, Aspergillus carneus
  mat_peptide (1)..(1007)
AQNHTDSEWPLHDNGLNTVVQWDHYSFQVHGQRIFVFSGEFHYWRIPVPGLWRDILEKIKAAGFTAFAFYSSWAYHAPNNHTVDFSTGARDITPIYELAKELGMYIIVRPGPYVNAEASAGGYPLWVTTGAYGSLRNDDARYTEAWKPYFAKMSEITSQYQVTDGHNTFCYQIENEYGQQWIGDPVDRNPNQTAVAYMELLEESARENGIVVPLTANDPNMNTKSWGNDWSNAGGNVDVVGLDSYPSCWTCDVTQCTSTNGEYVPYKVMGYYDYFQEVQPTMPGFMPEFQGGSYNPWAGPEGGCPGDTGVDFANLFYRWNIAQRVTAMSLYMLYGGTNWGAIAAPVTATSYDYSSPISEDRSIGSKYYETKLLALFTRSATDLTMTDRIGNGTQYTNNPAVAAYELRNPVTNGAFYVTIHADSTVGSDESFRLNVNTSAGAFTVPSKGAIRLNGHQSKIVVTDFRFGPSHSLLYSTAEVLTHAVFDKQATIVLWVPTGESGEFAVKGAKSGKVESCPRCSNATFTRKKDVLVVNFTQTGGMSVLQLNNGVRVVLLDRPAAYNFWAPPVTDDPFAPETDLVLVQGPYLVRSASLSGSTLALRGDSIKETALEIFAPKKVKTVTWNGKRVKTSKSSYGSLTASLAPPPAVTLPALTSTRWKSQDSLPERLPSYDDSGPAWVDADHMTTQNPRTPETLPVLYADEYGFHNGIRLWRGSFTDAASGVYLNVQGGAAFGWSAYLNGHFLGSHLGTATTSQANKTLVFPTGALNQNATNTLLVIHDDTGHDQTTGALNPRGILAARLLPASNAAADSTAPTFTRWRVAGTAGGESDLDPVRGVYNEDGLFAERVGWHLPGFDDGAWPAANTTAVAQETGTVSLSFTGATVRFFRTVIPLHLPRGIDASISFVLGTPAGTSTAYRAQLFVNGYQYGRYYPHIGNQVVYPVPAGVLDYDGENTIGVAVWAQSDAGAAINLDWRVNYVADSSLDAVRLTGEGSLRPQWSEARERYA

SEQ ID NO: 59 - DNA, 3317 bp, Penicillium quercetorum
  CDS (1)..(810)
  sig_peptide (1)..(69)
  mat_peptide (70)..(3314)
  CDS (876)..(1869)
  CDS (1923)..(2216)
  CDS (2273)..(2344)
  CDS (2400)..(2487)
  CDS (2540)..(3314)
atgacgcgggcaacgcgtctattctacggattgggcacgatcttctccctgctcggtgctacaattgccgcggagaaccaaacaactaccgaatggcccctgcacgatgatggtctgaaccaagtcgtccaatgggaccactacagcttccagatcaacagtcagcgcatcttcatcttctcgggtgaattccactactggcgcatccccgttcctggtctgtggcgcgatatcctcgagaagatcaaggcggtgggtttcacggcgtttgccttttactcgagctgggcctaccatgcgcccaacaaccagacgctggactttaccaccggcgcgcatgactttactcccctgtttgagttggcgaaggagcttggactgtacattattgttcgccctggaccgtatgtcaatgccgaagccagtgcgggtggcttcccgctgtggctgactacgggtgattatggtacgcttcgcaataatgatacgcgctatacgaaagcctggacgccgtacttcaccaagatgtcccagatcaccagcaagtaccaggtcactgatgggcagaacgcgattgtctatcagatcgagaacgagtacggggagcaatgggttggctcggcgtcgaagcgtgtgcccaatgaaaaggctatcaactatatggaacttctcgaggccaatgcccgtgccaatggtattactgtgccattgactgcaaacgatccgaacatgaactcgcactcgtggggaagtgattggtctaaggagggtggtaatgtggatgttgcgggagtagactcgtacccttcggtaagttcgctcatgtttgctttaaatcatgactctggaagactgatgagcctgaatgaaaatagtgctggacctgcgacctcagccaatgtacctccaccaatggcgaatacatcccgttccaggtcatggactactacgattacttccaagagtcgcagccaaccatgcccgaattcatgcccgagttccagggtggttcatacaacccctggggtggtcctgaaggcggctgtgccgagaactcgaaccaggactttgcgaatctgttctaccggtggaacattggccaacgtgtcacagcgatgagcttatacatgctgttcggaggcacgaactggggtgcgattgcggcgcccgtcactggcagcagctacgattactcggctcctatctcagaggatcgatctatcggggacaagtactacgagaccaagctgctagctttgttcacgcgctgtgcgaaggacttgacgatgacgaacttgattggtaatgggactcagtatactgataatggcaatgtccgtgcctatgaactgcggaacccagacacgaacgccggtttctatgcgactttccacactaacacgtccgtctctaccaatgaagccttccatctcaaggtgaacacctctgctggtgccttgactgttcccacacatggcggtgtggttcgattgaacggacaccaatccaagattctggtgacggatttcacctttggaaaggagacgttgctgtattccaccgccgaggttttgacatatgccgtgtttgataagactcccacgctggttctgtggatgccgacgggtgaaacgggcgagttcaatatcaagggcgcaaagaagggatcggtccagaagtgtcagggatgctctagtgtgaagttcttcaaggagcacggcggtctgactgccgccattacccagtcttctggcatgagtgtgctggcgattgacgacatccaagtgattgtccttgacagaacatctgcgtataaattctgggctccggcgcttacgaatgacccgcttgtgcccgagacggagagtggtaagttacactacttgtagcgacttttcataccaaatctaaccatctggcagtgcttgttcaaggaccttatctcgttcgcggcgcttctctctcgggctcgaagcttgctgttacaggtgatattatcaacgctacgacactggaggtctttgccccgaaggctgttaagtctattacttggaatggaaagacccttaaaactcaacgtaccgagtatggtagtctgaaggggtccattgcggcacccaaggctgttactctaccctctttcaaatcctggaagtccaaagacagtcttcctgagcgtttggctgactatgatgatgcgggagctgcgtgggttggtaagaattgcctgttcttgacacacagcctatcattcatctaactgtccttctagatgcaaaccaccagtccacattgaaccctcgtgcccctactactctgccagtcatgtacgcagatgaatacggtaagcgctcccttcaatgcacacgtctagccaataatctgacagccatatccaggcttccacaacggcgtccgcctgtggcgcggatacttcaacggctctgcaacaggggcctacatcaacgtccagggtggatatgccttgtaagtccctctactcgaaccccaacccatgcccagcactaacacaatccagcggctggtccgcctggctcaacggccaattcatcggctcctacctcggctccgccgacctcgagtccggcaacctatccctatccttcaccaacgcaaccatcaacaccaacaaacccaacatcctcctcatcgtccatgacgacacaggccacgacgagacaagcggcgccctcaatccccgcggtatcctcgacgcccacctcctcggctcatcatccggcttcacccactggcgtctcgccggtaccgcgggcggcgagtccaacctcgaccccgtgcgcggcgtcttcaacgaagatgggctctacggcgaacgggttggctggcatctcccgggctacgacgactcgacctggtccagcagcggtggttcaagtctaagcttcactggcgcaacagtccgcttcttccgcacaaccatcccgctcaatttcccctccaacacagacgtatcaatctccttcatcttgtccacaccgtctggcagcacgaccgcataccgggcccagatctttgtgaacgggtaccagtacggccggtataacccgtacatcgggaaccaggtggtgtatcctgttccggcggggattttgaactacagcggggagaatacggtggctgttgctgtgtgggcgcagacggaggagggggcgaggatggaggtggattggcgggtgaattatgtggcggatagttcgttggatgttgttagtgttagtaagaaggcggaggggttgaggacgaagtggactgaggtgcgggagaagtttgcttga

SEQ ID NO: 60 - protein, 1011 aa, Penicillium quercetorum
MTRATRLFYGLGTIFSLLGATIAAENQTTTEWPLHDDGLNQVVQWDHYSFQINSQRIFIFSGEFHYWRIPVPGLWRDILEKIKAVGFTAFAFYSSWAYHAPNNQTLDFTTGAHDFTPLFELAKELGLYIIVRPGPYVNAEASAGGFPLWLTTGDYGTLRNNDTRYTKAWTPYFTKMSQITSKYQVTDGQNAIVYQIENEYGEQWVGSASKRVPNEKAINYMELLEANARANGITVPLTANDPNMNSHSWGSDWSKEGGNVDVAGVDSYPSCWTCDLSQCTSTNGEYIPFQVMDYYDYFQESQPTMPEFMPEFQGGSYNPWGGPEGGCAENSNQDFANLFYRWNIGQRVTAMSLYMLFGGTNWGAIAAPVTGSSYDYSAPISEDRSIGDKYYETKLLALFTRCAKDLTMTNLIGNGTQYTDNGNVRAYELRNPDTNAGFYATFHTNTSVSTNEAFHLKVNTSAGALTVPTHGGVVRLNGHQSKILVTDFTFGKETLLYSTAEVLTYAVFDKTPTLVLWMPTGETGEFNIKGAKKGSVQKCQGCSSVKFFKEHGGLTAAITQSSGMSVLAIDDIQVIVLDRTSAYKFWAPALTNDPLVPETESVLVQGPYLVRGASLSGSKLAVTGDIINATTLEVFAPKAVKSITWNGKTLKTQRTEYGSLKGSIAAPKAVTLPSFKSWKSKDSLPERLADYDDAGAAWVDANHQSTLNPRAPTTLPVMYADEYGFHNGVRLWRGYFNGSATGAYINVQGGYAFGWSAWLNGQFIGSYLGSADLESGNLSLSFTNATINTNKPNILLIVHDDTGHDETSGALNPRGILDAHLLGSSSGFTHWRLAGTAGGESNLDPVRGVFNEDGLYGERVGWHLPGYDDSTWSSSGGSSLSFTGATVRFFRTTIPLNFPSNTDVSISFILSTPSGSTTAYRAQIFVNGYQYGRYNPYIGNQVVYPVPAGILNYSGENTVAVAVWAQTEEGARMEVDWRVNYVADSSLDVVSVSKKAEGLRTKWTEVREKFA

SEQ ID NO: 61 - protein, 988 aa, Penicillium quercetorum
  mat_peptide (1)..(988)
AENQTTTEWPLHDDGLNQVVQWDHYSFQINSQRIFIFSGEFHYWRIPVPGLWRDILEKIKAVGFTAFAFYSSWAYHAPNNQTLDFTTGAHDFTPLFELAKELGLYIIVRPGPYVNAEASAGGFPLWLTTGDYGTLRNNDTRYTKAWTPYFTKMSQITSKYQVTDGQNAIVYQIENEYGEQWVGSASKRVPNEKAINYMELLEANARANGITVPLTANDPNMNSHSWGSDWSKEGGNVDVAGVDSYPSCWTCDLSQCTSTNGEYIPFQVMDYYDYFQESQPTMPEFMPEFQGGSYNPWGGPEGGCAENSNQDFANLFYRWNIGQRVTAMSLYMLFGGTNWGAIAAPVTGSSYDYSAPISEDRSIGDKYYETKLLALFTRCAKDLTMTNLIGNGTQYTDNGNVRAYELRNPDTNAGFYATFHTNTSVSTNEAFHLKVNTSAGALTVPTHGGVVRLNGHQSKILVTDFTFGKETLLYSTAEVLTYAVFDKTPTLVLWMPTGETGEFNIKGAKKGSVQKCQGCSSVKFFKEHGGLTAAITQSSGMSVLAIDDIQVIVLDRTSAYKFWAPALTNDPLVPETESVLVQGPYLVRGASLSGSKLAVTGDIINATTLEVFAPKAVKSITWNGKTLKTQRTEYGSLKGSIAAPKAVTLPSFKSWKSKDSLPERLADYDDAGAAWVDANHQSTLNPRAPTTLPVMYADEYGFHNGVRLWRGYFNGSATGAYINVQGGYAFGWSAWLNGQFIGSYLGSADLESGNLSLSFTNATINTNKPNILLIVHDDTGHDETSGALNPRGILDAHLLGSSSGFTHWRLAGTAGGESNLDPVRGVFNEDGLYGERVGWHLPGYDDSTWSSSGGSSLSFTGATVRFFRTTIPLNFPSNTDVSISFILSTPSGSTTAYRAQIFVNGYQYGRYNPYIGNQVVYPVPAGILNYSGENTVAVAVWAQTEEGARMEVDWRVNYVADSSLDVVSVSKKAEGLRTKWTEVREKFA

SEQ ID NO: 62 - protein, 331 aa, Humicola insolens
  mat_peptide (1)..(331)
LQYKGVDWSSVMVEERAGVRYKNVNGQEKPLEYILAENGVNMVRQRVWVNPWDGNYNLDYNIQLARRAKAAGLGLYINFHYSDTWADPAHQTTPAGWPSDINNLAWKLYNYTLDSMNRFADAGIQVDIVSIGNEITQGLLWPLGKTNNWYNIARLLHSAAWGVKDSRLNPKPKIMVHLDNGWNWDTQNWWYTNVLSQGPFEMSDFDMMGVSFYPFYSASATLDSLRRSLNNMVSRWGKEVAVVETNWPTSCPYPRYQFPADVRNVPFSAAGQTQYIQSVANVVSSVSKGVGLFYWEPAWIHNANLGSSCADNTMFTPSGQALSSLSVFHRI

SEQ ID NO: 63 - protein, 332 aa, Myceliophthora thermophile
  mat_peptide (1)..(332)
ALTYRGVDWSSVVVEERAGVSYKNTNGNAQPLENILAANGVNTVRQRVWVNPADGNYNLDYNIAIAKRAKAAGLGVYIDFHYSDTWADPAHQTMPAGWPSDIDNLSWKLYNYTLDAANKLQNAGIQPTIVSIGNEIRAGLLWPTGRTENWANIARLLHSAAWGIKDSSLSPKPKIMIHLDNGWDWGTQNWWYTNVLKQGTLELSDFDMMGVSFYPFYSSSATLSALKSSLDNMAKTWNKEIAVVETNWPISCPNPRYSFPSDVKNIPFSPEGQTTFITNVANIVSSVSRGVGLFYWEPAWIHNANLGSSCADNTMFSQSGQALSSLSVFQRI

SEQ ID NO: 64 - protein, 324 aa, Meripilus giganteus
  mat_peptide (1)..(324)
LTYKGADISSVPLVEQAGIKYTDGGKVTPFENIIHNHGANTVRIRIWTAGDYNLQYGLALAKRVKAAGLTLVVDLHYSDTWADPGKQAIPSAWPKDLDGLNTQIWQYTKDVVTSFANQGTPIDILQVGNEINNGLLWPVGEISSNGINPVSQLLHSAINGAKAAGNPKILIHLANGWDWSGLNSFFGKVFIPGALSADEVDIIGVSFYPFYDAGATLSALKSSLANLANTFKKPIVVAETDWPVACSGVKLTEPSVPVSTSGQQTWIGDIKNVLQSLPNGLGQGIFYWEPGWIGNANLGSGCSDNLLVSSNGATRDSINIFNQM

SEQ ID NO: 65 - protein, 12 aa, Artificial Sequence
  SEQ ID NO: 65 is the conserved motif GV[T/M]PD[W/M]VQ[I/V]GNE.
  misc_feature (3)..(3): The amino acid in position 3 of the conserved motif is either threonine (T) or methionine (M).
  misc_feature (6)..(6): The amino acid in position 6 of the conserved motif is either tryptophan (W) or methionine (M).
  misc_feature (9)..(9): The amino acid in position 9 of the conserved motif is either isoleucine (I) or valine (V).
GVXPDXVQXGNE

SEQ ID NO: 66 - protein, 13 aa, Artificial Sequence
  SEQ ID NO: 66 is the conserved motif WADP[A/G]xQxKPxAW.
  misc_feature (5)..(5): The amino acid in position 5 of the conserved motif is either alanine (A) or glycine (G).
  misc_feature (6)..(6): The amino acid in position 6 of the conserved motif is any amino acid.
  misc_feature (8)..(8): The amino acid in position 8 of the conserved motif is any amino acid.
  misc_feature (11)..(11): The amino acid in position 11 of the conserved motif is any amino acid.
WADPXXQXKPXAW

SEQ ID NO: 67 - protein, 27 aa, Bacillus clausii
MKKPLGKIVASTALLISVAFSSSIASA

SEQ ID NO: 68 - DNA, 3138 bp, Penicillium simplicissimum
  CDS (1)..(235)
  sig_peptide (1)..(63)
  mat_peptide (64)..(3135)
  CDS (306)..(1382)
  CDS (1439)..(1940)
  CDS (2001)..(3135)
atgcggtttttcgcatttctcccgttgctccttatcggggcgctgtcgagcattgtctctgcgacggacaatggcaagactaccgatgttacttgggacaagtatagtctctccgtgaagggggagagagtctttgtcttttctggtgaattccattatatgcgtcttcctgttccggagatgtggcttgatgtgttccaaaagttgcgctccaatggcttcaacgcggtatccagtgagtaaaccaatatatatcccatacaccacactcaatcaattaaaaccaattcaactaaccgttcaagtctacttcttctggagcttccactccgcttcggaagacacatttgactttgaaaacggcgcccacgatgtccagcgcgtcttcgactacgctaaacaagccggtctgtatgtgattgcccgtgcaggaccctacatcaacgctgaaacctcggccggtggattcgccctgtgggcagcgaacggacaaatgggcagtgaacgaaccagtgcctcgtcctactacgacaaatggcttccctggatcctgaagatcggcaagatcatcgcggataaccagatcaccaacggcggaccggtgatcctgaaccagcacgagaacgagctccaggagaccacccacagcgcgaccaacactctagttctgtacatggagcaaatcgcagccgcattcgaggaggccggtgtcatcgtgcccagctcgcacaacgaaaaaggtatgcgctcggaaagctggtcgacagattacgaagacgtcggcggtgcagtaaacgtctacggcctcgattcataccccggcggtctgtcctgcacaaaccccgactcgggattcaacctcgtccgcacttactaccaatggttccagaactactcctacacacagcccgaattcctccccgaatttgagggcggctggttccagccctggggtggatatttctacgacgagtgtgccgcagagcactcgcccgaattcgccgacgtctattacaagaataacattgggtcccgggtcaccctgcagagtctgtatatggcctttggcgggacgaattggggtcatagtgccacgccggtcgtttatacttcgtatgactatgcggcgccgctaagggagacgagagagatccaggataaactcaagcagactaagttgattggtttgtttactcgggtttcatcgggattgttgcagactgtcatggagggcaatggaacgggatatactagtgatactagtatttatacgtgggctttgcggaatcccgagacggacgctgggttctatgtgcttgcgcatagtacgagttcgtctcgtgcggtgacgacgttctcgctgaatgttaatacttcggctggtatggttcctcacgctggagtgctttgagaatattttgactaactcgcttcttaggtgctctgactatccctgacattgaactggatggtcgccaaagcaaaatcatcgtcacggattacgaaatcggcaaggcctcgagccttctctactcatccgccgaggttctgacctacgctaccctcgacgtggacgtgctggtgctctacctgaacattggacaaaagggcgtgttcgcattcaagaatgccccatcccacttgacgttcaagacatacggtaactcgaacttgacttccaccacatcgaccaatggaacgcagtactcgtacacccaaggagatggtgcgaccgctgtcaagttctccaacggggttcttctatatctgctggacaaggaaaccgcttggaacttctttgctgtgactaccacgtccaacccgaatgtgacccccagcgaacacattcttgctcttggaccgtatttggttcgtgaggcgagtatcagccatgataccgttagcctgattggtgataatgcgaataccaccacactggagtaagttgattcccatggaagggtatttggtggaactgcacttgctaacctttctcatagagtctaccctggtaacgcccaggtaaccaagatcaagtggaatggcaaaccgattgcgactaagaagaccgcatacggcagtctcatcggctcagcccaaggcgcagaaaccgccaagatctccctgccctctctgacatcctggaagtctcaagatactcttcccgagatcaagcaagactacgacgactcgcgctggacggtctgcaacaagagcacgacggtcaactctgtcgcaccactgtcgctgcccgtcctatactcgggcgactacggataccacgcaggcaccaagatctaccgcggtcgcttcgacggacgcaatgccaccggcgccaacgtgacggtgcaaaacggcgtcgccgctggctgggcagcctggttgaacggcgactatgttggcggtgccctaggcaatccagctctcgcagcaacctccgacttgttaaccttcaacagctcctccctccgggataccgataacgtcctcacggtcgtgatggactataccggccacgacgagaacaacgtcaagccggccggtacccagaacccccgcggtatcttgggagccaccctcttcggcggcggcaacttcacctcctggcgcatccaaggcaacgcaggcggcgaagcaaacatcgaccccgtccgcggccccatgaacgaaggtggcctctacggcgaacgactcggctggcatctcccgggatacaccgcacccaagagcgcgggcagctcatcccccctgcagggtgtctcgaacgccgcaggacgcttctacacgacaaccttcaagctcaatctagaggccgatctggacgtcccgattggcctgcagctcggggcagcggccaataccagtgcggtggtgcaggtgtttatgaacgggtaccagtttggccattacctgccgcatattggaccgcagacgctgttcccgttcccaccgggtattatcaataatcggggggagaatacgttggcgattagtctgtgggcgttgacggatgagggggcggcgttggatcaggtggagttggtcgcgtacggggcgtatcggaccgggttcgattttaatcaggattggacgtacctgcagccgaagtggaagaataatcgggggtcgtatgtgtag

SEQ ID NO: 69 - protein, 983 aa, Penicillium simplicissimum
MRFFAFLPLLLIGALSSIVSATDNGKTTDVTWDKYSLSVKGERVFVFSGEFHYMRLPVPEMWLDVFQKLRSNGFNAVSIYFFWSFHSASEDTFDFENGAHDVQRVFDYAKQAGLYVIARAGPYINAETSAGGFALWAANGQMGSERTSASSYYDKWLPWILKIGKIIADNQITNGGPVILNQHENELQETTHSATNTLVLYMEQIAAAFEEAGVIVPSSHNEKGMRSESWSTDYEDVGGAVNVYGLDSYPGGLSCTNPDSGFNLVRTYYQWFQNYSYTQPEFLPEFEGGWFQPWGGYFYDECAAEHSPEFADVYYKNNIGSRVTLQSLYMAFGGTNWGHSATPVVYTSYDYAAPLRETREIQDKLKQTKLIGLFTRVSSGLLQTVMEGNGTGYTSDTSIYTWALRNPETDAGFYVLAHSTSSSRAVTTFSLNVNTSAGALTIPDIELDGRQSKIIVTDYEIGKASSLLYSSAEVLTYATLDVDVLVLYLNIGQKGVFAFKNAPSHLTFKTYGNSNLTSTTSTNGTQYSYTQGDGATAVKFSNGVLLYLLDKETAWNFFAVTTTSNPNVTPSEHILALGPYLVREASISHDTVSLIGDNANTTTLEVYPGNAQVTKIKWNGKPIATKKTAYGSLIGSAQGAETAKISLPSLTSWKSQDTLPEIKQDYDDSRWTVCNKSTTVNSVAPLSLPVLYSGDYGYHAGTKIYRGRFDGRNATGANVTVQNGVAAGWAAWLNGDYVGGALGNPALAATSDLLTFNSSSLRDTDNVLTVVMDYTGHDENNVKPAGTQNPRGILGATLFGGGNFTSWRIQGNAGGEANIDPVRGPMNEGGLYGERLGWHLPGYTAPKSAGSSSPLQGVSNAAGRFYTTTFKLNLEADLDVPIGLQLGAAANTSAVVQVFMNGYQFGHYLPHIGPQTLFPFPPGIINNRGENTLAISLWALTDEGAALDQVELVAYGAYRTGFDFNQDWTYLQPKWKNNRGSYV

SEQ ID NO: 70 - protein, 962 aa, Penicillium simplicissimum
  mat_peptide (1)..(962)
TDNGKTTDVTWDKYSLSVKGERVFVFSGEFHYMRLPVPEMWLDVFQKLRSNGFNAVSIYFFWSFHSASEDTFDFENGAHDVQRVFDYAKQAGLYVIARAGPYINAETSAGGFALWAANGQMGSERTSASSYYDKWLPWILKIGKIIADNQITNGGPVILNQHENELQETTHSATNTLVLYMEQIAAAFEEAGVIVPSSHNEKGMRSESWSTDYEDVGGAVNVYGLDSYPGGLSCTNPDSGFNLVRTYYQWFQNYSYTQPEFLPEFEGGWFQPWGGYFYDECAAEHSPEFADVYYKNNIGSRVTLQSLYMAFGGTNWGHSATPVVYTSYDYAAPLRETREIQDKLKQTKLIGLFTRVSSGLLQTVMEGNGTGYTSDTSIYTWALRNPETDAGFYVLAHSTSSSRAVTTFSLNVNTSAGALTIPDIELDGRQSKIIVTDYEIGKASSLLYSSAEVLTYATLDVDVLVLYLNIGQKGVFAFKNAPSHLTFKTYGNSNLTSTTSTNGTQYSYTQGDGATAVKFSNGVLLYLLDKETAWNFFAVTTTSNPNVTPSEHILALGPYLVREASISHDTVSLIGDNANTTTLEVYPGNAQVTKIKWNGKPIATKKTAYGSLIGSAQGAETAKISLPSLTSWKSQDTLPEIKQDYDDSRWTVCNKSTTVNSVAPLSLPVLYSGDYGYHAGTKIYRGRFDGRNATGANVTVQNGVAAGWAAWLNGDYVGGALGNPALAATSDLLTFNSSSLRDTDNVLTVVMDYTGHDENNVKPAGTQNPRGILGATLFGGGNFTSWRIQGNAGGEANIDPVRGPMNEGGLYGERLGWHLPGYTAPKSAGSSSPLQGVSNAAGRFYTTTFKLNLEADLDVPIGLQLGAAANTSAVVQVFMNGYQFGHYLPHIGPQTLFPFPPGIINNRGENTLAISLWALTDEGAALDQVELVAYGAYRTGFDFNQDWTYLQPKWKNNRGSYV

SEQ ID NO: 71 - DNA, 3309 bp, Aspergillus westerdijkiae
  CDS (1)..(801)
  sig_peptide (1)..(60)
  mat_peptide (61)..(3306)
  CDS (852)..(1848)
  CDS (1898)..(2191)
  CDS (2239)..(2310)
  CDS (2360)..(2447)
  CDS (2499)..(3306)
atggcgcgcatcatgcaccttgccgtgctgcttctttccagcatcggactgctggctgctgcccagaatcagtccgactctgactggcctctgcacgacaacggtctgaacaccgccgtgcaatgggaccattacagcttccatgtccacggacagcgcatcttcatcttctccggcgagtttcactactggcgtattcccgtccccgagctttggcgcgacatcctcgagaaggtcaaagccaccggcttcaccgcgtttgccttctactctagctgggcgtaccatgcgccgaacaaccacacggtggacttccacaccggtgcgcgcgacatcacgcccatcttcgagctcgccaaggagctgggcatgtatatgatcgtgcggcccgggccgtatgtcaatgccgaggccagcgctggtggctttccgctgtgggcgaccaccggtgcgtatgggtcgatgcgcaatgacgaccccaggtatactgcggcgtggaagccgtactttgagaagatgtcgcaaatcaccagtcagtaccagatcaccgatggggaaaacactttctgctatcagatcgagaacgagtatggccagcagtgggttggtgatccccgtgatcggaacccgaataagactgcggtcgcctatatggaactgctcgaggagagtgcccgtgagaatggtattgtcgtgccgctgacggccaacgatccgaacctgaacacccgctcttggggaaacgactggtccaacgctggaggaaacgttgacgttcctggagtggattcgtatccctcagtgagttacctaaatcacatctgggtaatgcaaattactaatctttccagtgctggacttgtgatgtctctcaatgcacctccaccaacggagagtacgttccttacaaagtgatcccctattacgactacttccaggaggtccagccctcgatgcctgccttcatgcccgaattccagggtggatcttacaacccctgggccggccccgaaggtggatgtcccgaggataccggagcggactttgccaacctgttctaccggtggaacatcgcccagcgagtgaccgccatgagcttgtacatggtatttggcggaaccaactggggctcgctggctgcccccgttacagccaccagctacgactactcctccccgattgccgaagaccgctcgattggtgacaagtactacgagaccaagctgctttccctgttcactcgtagcgccaaggatctcaccatgaccgacctcatcggcaacggcaccaagtacaccgacaatgctgccgtcagcgcgtacgaactccggaaccccgagaccaacggtgccttctacgtcaccatccacaaggacaccaccgtcggctcggacgagtccttcaagctccacgtgaacacctccgctggcgcgctgactatcccaagcgagggggcaaagatccgcctgaacggccatcagtccaagatcatcgtgactgactttgccttcggctctaagaccctcctgtactccaccgccgaggtgttgacctatgcggtcatcgatgaccagcctactctggtgctttgggtcccgaagggagaatctggcgagttcgctgtcaagggcactaagtctggcaaggtggcgagctgcaacggctgctccagcgtcaagttcaacggaaagaaggaccacgtggttgttgggttcacacaggccaagggcatgagcgtgtatcagctggatgatgatgtccgtgtcgttgttctcgaccggtcgtccgcttatcacttctgggcccctactttgactgatgatccgattgccccggaggatgaaattggtatgctcccgtgtccgagagaaatgactgattgctaatatcatactagtcctggtcgagggcccctacctcgtccgctcggccagcgtcgagggatctacccttgctctccgcggtgactctaccgacaagaccaacctggaggttttcgctcctaagagcgtcaagaccatcacctggaatggcaagaaggtcaagtcctccgagacctcctatggcagcctcaaggccacgctcgccgcgccaccctcgattaagctaccctctttcggctcatggcggtcgaacgacagcttgccggagcgcttggagtcgtacgatgactctggcccggcctgggttggtaagtacatctccacggcggtccaagattcccgctcaccagaacagatgccaaccatgaaaccacgctgaacccgcatccccctgtcacgactcctgtcttgtacgcaaacgaatacggtatgcatctctggccttcattctttagtctcatgctcatcacgtccaggcttccacaacggcgtccgcctctggcgcggctatttcaacggaaccgcctccggcgtcttcctcaacatccaaggtggcgctgcattgtaagcaccctctccctcctaacatccacgaccatctaaccaaaagtccagcggctggtccgcctatctcaacggccacttccttggctcctacctcggcaacgccaccatcgcgcaagccaacaaaaccctcaccttcccgaacaacacgctccacacgcgccccggctcccggaacaccctcctcgtcatccacgacgacaccggccacgaccagaccaccggcgtgctcaacccgcgcggcatcatcgaagcccgcctcctcggctccaacgccccgaacttcacccactggcgtctcgccggtaccgccggcggcgaatcaaacctcgatcccgtccgcggcgtctacaacgaagacggcctccacgcggagcgcgtcggctggcatctccctggcttcgacgacagcgactggcctgtcaccaaccactcctcctcctcctctagctccaaatccctctccaccctctccttcaccggcgcaaccgttcgcttcttccgcaccaccatccccctaaatatcccctcgggcctcgacgtctcgatctccttcctcctcggcacgccgacaggcacgagtaaggcctaccgcgcgcagctcttcgttaacggctaccagtacgggcgctactatccgcacatcggcaaccaggtcgtgtatccggtcccggcggggattttggattaccgcggcgagaacacgatcgggttggctgtttgggcgcagagcgaggatggcgcggcggtcagtgttgattggagggtgaattatgtggcggatagttcgttggatgttgcggggattggggaggagaggttgaggccggggtatgagaaggtgagggagaagtttgcttga

SEQ ID NO: 72 - protein, 1020 aa, Aspergillus westerdijkiae
MARIMHLAVLLLSSIGLLAAAQNQSDSDWPLHDNGLNTAVQWDHYSFHVHGQRIFIFSGEFHYWRIPVPELWRDILEKVKATGFTAFAFYSSWAYHAPNNHTVDFHTGARDITPIFELAKELGMYMIVRPGPYVNAEASAGGFPLWATTGAYGSMRNDDPRYTAAWKPYFEKMSQITSQYQITDGENTFCYQIENEYGQQWVGDPRDRNPNKTAVAYMELLEESARENGIVVPLTANDPNLNTRSWGNDWSNAGGNVDVPGVDSYPSCWTCDVSQCTSTNGEYVPYKVIPYYDYFQEVQPSMPAFMPEFQGGSYNPWAGPEGGCPEDTGADFANLFYRWNIAQRVTAMSLYMVFGGTNWGSLAAPVTATSYDYSSPIAEDRSIGDKYYETKLLSLFTRSAKDLTMTDLIGNGTKYTDNAAVSAYELRNPETNGAFYVTIHKDTTVGSDESFKLHVNTSAGALTIPSEGAKIRLNGHQSKIIVTDFAFGSKTLLYSTAEVLTYAVIDDQPTLVLWVPKGESGEFAVKGTKSGKVASCNGCSSVKFNGKKDHVVVGFTQAKGMSVYQLDDDVRVVVLDRSSAYHFWAPTLTDDPIAPEDEIVLVEGPYLVRSASVEGSTLALRGDSTDKTNLEVFAPKSVKTITWNGKKVKSSETSYGSLKATLAAPPSIKLPSFGSWRSNDSLPERLESYDDSGPAWVDANHETTLNPHPPVTTPVLYANEYGFHNGVRLWRGYFNGTASGVFLNIQGGAAFGWSAYLNGHFLGSYLGNATIAQANKTLTFPNNTLHTRPGSRNTLLVIHDDTGHDQTTGVLNPRGIIEARLLGSNAPNFTHWRLAGTAGGESNLDPVRGVYNEDGLHAERVGWHLPGFDDSDWPVTNHSSSSSSSKSLSTLSFTGATVRFFRTTIPLNIPSGLDVSISFLLGTPTGTSKAYRAQLFVNGYQYGRYYPHIGNQVVYPVPAGILDYRGENTIGLAVWAQSEDGAAVSVDWRVNYVADSSLDVAGIGEERLRPGYEKVREKFA

SEQ ID NO: 73 - protein, 1000 aa, Aspergillus westerdijkiae
  mat_peptide (1)..(1000)
AQNQSDSDWPLHDNGLNTAVQWDHYSFHVHGQRIFIFSGEFHYWRIPVPELWRDILEKVKATGFTAFAFYSSWAYHAPNNHTVDFHTGARDITPIFELAKELGMYMIVRPGPYVNAEASAGGFPLWATTGAYGSMRNDDPRYTAAWKPYFEKMSQITSQYQITDGENTFCYQIENEYGQQWVGDPRDRNPNKTAVAYMELLEESARENGIVVPLTANDPNLNTRSWGNDWSNAGGNVDVPGVDSYPSCWTCDVSQCTSTNGEYVPYKVIPYYDYFQEVQPSMPAFMPEFQGGSYNPWAGPEGGCPEDTGADFANLFYRWNIAQRVTAMSLYMVFGGTNWGSLAAPVTATSYDYSSPIAEDRSIGDKYYETKLLSLFTRSAKDLTMTDLIGNGTKYTDNAAVSAYELRNPETNGAFYVTIHKDTTVGSDESFKLHVNTSAGALTIPSEGAKIRLNGHQSKIIVTDFAFGSKTLLYSTAEVLTYAVIDDQPTLVLWVPKGESGEFAVKGTKSGKVASCNGCSSVKFNGKKDHVVVGFTQAKGMSVYQLDDDVRVVVLDRSSAYHFWAPTLTDDPIAPEDEIVLVEGPYLVRSASVEGSTLALRGDSTDKTNLEVFAPKSVKTITWNGKKVKSSETSYGSLKATLAAPPSIKLPSFGSWRSNDSLPERLESYDDSGPAWVDANHETTLNPHPPVTTPVLYANEYGFHNGVRLWRGYFNGTASGVFLNIQGGAAFGWSAYLNGHFLGSYLGNATIAQANKTLTFPNNTLHTRPGSRNTLLVIHDDTGHDQTTGVLNPRGIIEARLLGSNAPNFTHWRLAGTAGGESNLDPVRGVYNEDGLHAERVGWHLPGFDDSDWPVTNHSSSSSSSKSLSTLSFTGATVRFFRTTIPLNIPSGLDVSISFLLGTPTGTSKAYRAQLFVNGYQYGRYYPHIGNQVVYPVPAGILDYRGENTIGLAVWAQSEDGAAVSVDWRVNYVADSSLDVAGIGEERLRPGYEKVREKFA

SEQ ID NO: 74 - DNA, 3299 bp, Aspergillus wentii
  CDS (1)..(789)
  sig_peptide (1)..(60)
  mat_peptide (61)..(3296)
  CDS (836)..(1829)
  CDS (1877)..(2170)
  CDS (2220)..(2291)
  CDS (2339)..(2426)
  CDS (2474)..(3296)
atggcgcgcattttccatttgtttcttgccctactttcaagtatagggcttttggcagctgcagagtcacaatggcctctccacgataacagcttaaacaccgtcgttcaatgggatcattacagcttccagatccacgggcagagaatcttcgtcttctccggtgaattccactactggcgcattccagttccaggactatggagggatattcttgagaagattaaagcggctggatttactgcattcgcattttactccagttgggcttaccatgcgccaaataaccataccgttgacttttcgaccggtgctcgtgatatcacacctattttcgaacttgccaaggagttgggcttgtatatcatcgttcgcccagggccatatgtcaatgcggaagccaatgctggtggctttcccttgtggctgacgactggggaatacggaacgctacgcaatgacgatgaacgctatactgccgcgtggaagccgtacttcactaaaatgtcgcagattacgagcaaatatcagatcacggatggcgagaacaccttgttttatcagattgaaaacgaatacggagaccagtggatcggcgatccaagtgatcgagttccgaataatactgcaattgcttatatggagcttctcgaggcgagtgcacgggaaaacggcatcaatgtacctctcaccgcgaatgatcctaatatgaactcgaaatcttgggggaaagattggtctaatgctggtggaaacgttgacgcccctggcttggactcttacccgtcggtaggttaaccataactctaagactggattattctgacagtagcagtgttggacgtgtgatattagccaatgcacctcgacgaatggcgagtatgtgccgtacaaagtaatgcagtattacgactacttccaagaagttcaaccgacaacgccgtctttcatgcccgagttccagggcggttcttacaatccctgggcaggacctgaaggtggatgctccgagaataccggggcagactttgcgaatctgttctatcggtggaacattggccagcatgtgacggctatgagtctgtacatgctatacggaggtacgaattgggggtcgctcgctgcaccggtgacggcaagtagttatgactactcagccccgatttccgaagatcggtctattggggcaaagtattatgagactaaactactggcattgttcacgcggtgtgcaagagatttgaccatgactgaattgattggaaatggaactcagtataccgataatatagcagtggaagcatacgaattgaggaatccgcagaccaatgccggtttctacgttaccatccacagcaactcttcctctgggacaaacgaggcctttcaacttcaggtcaacacttctgtcggaggtctgactgttcctagccatggaggtactatacgtctcaatggtcaccagtccaagattatcgtgacggactttacatttggttccaagactcttctctattccaccgcggaggttctcacctacgctgtgttggatgacaaacctacacttgtcctctgggtacctaccggagaatccggcgagttctccatcaaaggagtcaagtctggatcagtcagtaactgtcagggctgctcgggtatgggtttctaccaggaaaatggtggtctcacggtaagattcacccagtcatctggaatgagcatcctccagctcgacgatgtacgcgtggttttactcgatagaacaagcgcatataatttctgggcgcctgcattgacaaatgacccatttgttccagagacagaaagtggtatgtttcgcctgatttattaattggcatttactaaccggtcgaagttctgattcaaggtccatacctcgttcgcggtgccaaaattactgaatcaactcttgcagtgactggtgattctgtggatgctacgagtatcgaggtcttcgcaccccagaccttggatacaatcacctggaatggcaaagaggtcaaaaccacgaggacggaatatggaagtctgcgggcttctcttgctgcaccaccatctattaagttaccctcgttgacatcgtggaaaacaaaagacagtctaccagagcggttgccatcatatgatgactctggtgaggcgtgggctggtaagtgccacttatctatctacactcactcaatgctaatcgaggatagatgccaaccatatgacaacttcgaatccacataaaccagaaacttatcccgttctttatggggatgattatggtatgtccattgtatccatgatagttatcaataagctaacaaagaaggcttccacaacggcatccgtctctggcgaggatactttaacaacaccgcgaaaggcgtctacctgaacatccaaggaggaacagctttgtaagatccatctcttttccatttaggtgaacaagctaacaaatcagtggctggtctgcctatctgaacggccacttcctctcctcttacctgggcaatgcaacagaaacccaaggaaataagaccatcctcttcccatctgatatcctctccacaaaaccagaaacgaatccaaataccctcctcatcatccacgatgacacaggccacgaccaaacaaccggcgttctcaacccgcgcggcatcctcgaagcacgtctcctcgacgaagacgagaaaagcagtgaagacctcgcatttacgcactggcgcgttgcaggtacagctggaggagaatcgaatctcgatcccgtccgcggcgtatacaatgaagacggactatacgccgaacggatgggctggcatttacccggtttcgacgatagtgattggtctacgattaacacaaccacgtccagtactaccagcagccccccattaacattcaccaacgcaaccatccaattcttccgaagcgtcatccccctcgacctccccaacaacaccgacacatccatgtccttcatcctctccactccatccaccagcagcaaagcctaccgcgcccaaatattcataaacgggtaccaatacggccggtacaacccccacatcgggaaccaggtggtcttccccgttccgccggggatactggattaccacggcgacaacacgattggagtagcggtgtgggcacagagcgaggatggggcgagtattgaattagattggagggtgaattacgttgctgatagttcgctggatgtgggccgtttggatgaggggggatcgctgaggccggggtggagtgaggagaggttgaggtttgcgtga

SEQ ID NO: 75 - protein, 1020 aa, Aspergillus wentii
MARIFHLFLALLSSIGLLAAAESQWPLHDNSLNTVVQWDHYSFQIHGQRIFVFSGEFHYWRIPVPGLWRDILEKIKAAGFTAFAFYSSWAYHAPNNHTVDFSTGARDITPIFELAKELGLYIIVRPGPYVNAEANAGGFPLWLTTGEYGTLRNDDERYTAAWKPYFTKMSQITSKYQITDGENTLFYQIENEYGDQWIGDPSDRVPNNTAIAYMELLEASARENGINVPLTANDPNMNSKSWGKDWSNAGGNVDAPGLDSYPSCWTCDISQCTSTNGEYVPYKVMQYYDYFQEVQPTTPSFMPEFQGGSYNPWAGPEGGCSENTGADFANLFYRWNIGQHVTAMSLYMLYGGTNWGSLAAPVTASSYDYSAPISEDRSIGAKYYETKLLALFTRCARDLTMTELIGNGTQYTDNIAVEAYELRNPQTNAGFYVTIHSNSSSGTNEAFQLQVNTSVGGLTVPSHGGTIRLNGHQSKIIVTDFTFGSKTLLYSTAEVLTYAVLDDKPTLVLWVPTGESGEFSIKGVKSGSVSNCQGCSGMGFYQENGGLTVRFTQSSGMSILQLDDVRVVLLDRTSAYNFWAPALTNDPFVPETESVLIQGPYLVRGAKITESTLAVTGDSVDATSIEVFAPQTLDTITWNGKEVKTTRTEYGSLRASLAAPPSIKLPSLTSWKTKDSLPERLPSYDDSGEAWADANHMTTSNPHKPETYPVLYGDDYGFHNGIRLWRGYFNNTAKGVYLNIQGGTAFGWSAYLNGHFLSSYLGNATETQGNKTILFPSDILSTKPETNPNTLLIIHDDTGHDQTTGVLNPRGILEARLLDEDEKSSEDLAFTHWRVAGTAGGESNLDPVRGVYNEDGLYAERMGWHLPGFDDSDWSTINTTTSSTTSSPPLTFTNATIQFFRSVIPLDLPNNTDTSMSFILSTPSTSSKAYRAQIFINGYQYGRYNPHIGNQVVFPVPPGILDYHGDNTIGVAVWAQSEDGASIELDWRVNYVADSSLDVGRLDEGGSLRPGWSEERLRFA

SEQ ID NO: 76 - protein, 1000 aa, Aspergillus wentii
  mat_peptide (1)..(1000)
AESQWPLHDNSLNTVVQWDHYSFQIHGQRIFVFSGEFHYWRIPVPGLWRDILEKIKAAGFTAFAFYSSWAYHAPNNHTVDFSTGARDITPIFELAKELGLYIIVRPGPYVNAEANAGGFPLWLTTGEYGTLRNDDERYTAAWKPYFTKMSQITSKYQITDGENTLFYQIENEYGDQWIGDPSDRVPNNTAIAYMELLEASARENGINVPLTANDPNMNSKSWGKDWSNAGGNVDAPGLDSYPSCWTCDISQCTSTNGEYVPYKVMQYYDYFQEVQPTTPSFMPEFQGGSYNPWAGPEGGCSENTGADFANLFYRWNIGQHVTAMSLYMLYGGTNWGSLAAPVTASSYDYSAPISEDRSIGAKYYETKLLALFTRCARDLTMTELIGNGTQYTDNIAVEAYELRNPQTNAGFYVTIHSNSSSGTNEAFQLQVNTSVGGLTVPSHGGTIRLNGHQSKIIVTDFTFGSKTLLYSTAEVLTYAVLDDKPTLVLWVPTGESGEFSIKGVKSGSVSNCQGCSGMGFYQENGGLTVRFTQSSGMSILQLDDVRVVLLDRTSAYNFWAPALTNDPFVPETESVLIQGPYLVRGAKITESTLAVTGDSVDATSIEVFAPQTLDTITWNGKEVKTTRTEYGSLRASLAAPPSIKLPSLTSWKTKDSLPERLPSYDDSGEAWADANHMTTSNPHKPETYPVLYGDDYGFHNGIRLWRGYFNNTAKGVYLNIQGGTAFGWSAYLNGHFLSSYLGNATETQGNKTILFPSDILSTKPETNPNTLLIIHDDTGHDQTTGVLNPRGILEARLLDEDEKSSEDLAFTHWRVAGTAGGESNLDPVRGVYNEDGLYAERMGWHLPGFDDSDWSTINTTTSSTTSSPPLTFTNATIQFFRSVIPLDLPNNTDTSMSFILSTPSTSSKAYRAQIFINGYQYGRYNPHIGNQVVFPVPPGILDYHGDNTIGVAVWAQSEDGASIELDWRVNYVADSSLDVGRLDEGGSLRPGWSEERLRFA

SEQ ID NO: 77 - DNA, 3310 bp, Aspergillus lentulus
  CDS (1)..(801)
  sig_peptide (1)..(60)
  mat_peptide (61)..(3307)
  CDS (851)..(1847)
  CDS (1899)..(2192)
  CDS (2246)..(2317)
  CDS (2367)..(2454)
  CDS (2518)..(3307)
atggcgcacatctaccaacttctccttcttcttctttcaaatctgtggttcgcgacagctgctcagaaccagtcagagactgaatggcctcttcatgataatggcttgagcaaggtagtgcaatgggaccactatagcttccacgtcaacgggcagaggatcttcgtcttttccggcgaattccattactggcgtattccagtccccgagttgtggagggatgttctcgagaaggtgaaagctaccggtttcactgcgtttgcgttctactctagctgggcctatcatgcgcccaacaaccacacggtcgacttctcgaccggcgctcgcgatatcacgcccatctttgagcttgcaaaggagctcggcatgtatatgattgtgcgccccgggccctacgtcaatgctgaagccagcgcgggcggcttccctctgtggctgacgactggcgagtatggctcgctgcggaatgatgacccgcggtatacggccgcatggacgccgtactttgccaacatgtcgcaaatcactagcaagtatcaggttacggatggacataacacgctcgtctaccagattgagaatgagtacggtcagcagtggatcggagatcccaaggatcgcaagccgaataagactgcggttgcttacatggagctcttggaagcatctgctcgtgagaatggtatcactgtgccattgacaagcaacgatcccaacatgaactcgaaatcttggggatcggactggtccaatgctggaggcaatgtcgacgtggctggtttggattcttatccgtcggtgagttaccattagatcctttttatttgtttcgttctgactgttgaagtgctggacatgcgacgtgagccaatgtacctccaccaatggggagtatgttccctacaaagtgattgattattacgactacttccaagaagttcagccaactcttccctcgttcatgcccgagttccagggcggttcgtacaacccctgggccggtcctgaaggtggatgtcctcaggacaccggcgccgagtttgctaacctgttctaccgatggaacattggccagcgagtgaccgccatgagtctgtatatgctgtacggaggaaccaactggggtgcaattgctgctcctgtgacagcaaccagctacgactactccgctcccatctccgaagaccgctcgattggagccaagtattccgagaccaagctactggcattgttcacccgtaccgcaaaggacctcacaatgacagaggcgatcgggaacggaacacaatataccaccaacacagccgtccgtgcattcgagttgagaaatcctcagaccaacgccgggttctacgtcacattccacaacgacaccaccgttggtggaaatcaagcgttcaaactccatgtcaacacttctgtcggtgccttgactgtccccaagaacgagggtgtgatccagctgaatggtcatcaatccaagatcatcgtgaccgacttcacgctcggcaaacgtactcttctctattcaactgccgaggtcttgacctacgccgtttttgaagacaggcccaccctcgtgctctgggttcctactggggaatccggcgagttcgcgatcaagggagccaagtcaggaaaggttgaaaatggcgatggctgctcgggaatcaaatttgagagtgagaagaactatctcgtcgtgaatttctctcaggccaagggattgagcgtcttgcggctcgataatggtgtgcgcgtggttctgctcgacaaggccgccgcgtaccgcttctgggctcctgcattgacaaatgatcctgtcgtgcaagaggccgaaactggtaagttcacttcatgcgtagtacattgtcatttcatactaatggttacagtgctcgtccacggcccgtaccttgttcgctccgccagcgtgtcgaagtccacactggcgctccgaggagactcagtcgagaagacgacactggaaatcttcgcacctcacagcgtgagggagattacctggaatgggaaacaagtgaagacctctcagacttcatatggcagtctcaaagcgactctcgctgcaccgccgaccataaagttacccgctctcacctcctggagatccaacgacagcttgccggagcggcttccatcgtatgacgattccggaccggcctggattggtgagttggattccaatcgatctggcctggacgaaatctaatgcgtttgacagaggcaaaccacatgaccacatctaaccccagtaaacctgcaacccttccagtcctatacgcagacgaatacggtatgtcaacctctataccgacaccatcacaagtctaacccgcctacaggcttccacaacggcgtccgcctctggcgcggctacttcaacggctctgcttccggagtctacctcaacatccaaggaggaagcgccttgtacgttaccctccccatcccctctcaactatctcatcgaaactaacaacctcccctccgcagcggctggtccgcctggctaaacggccacttcctcgactcccacctcggcgacgcaacaacctcccaagcaaacaaaaccctccccttcccaccctccctcctcaaccccaccgaaaacgtcctcctcatcgtccacgacgacacaggccacgaccagacaaccggcgccctaaacccacgcggcatcctcgcggcccgcctcctctccaacgactcctcgtcccccgcgccggaattcacccgctggcgcctcgccggcaccgcaggcggggaatcgaacctcgatcccatccgcggcgtcttcaacgaggacggcctcttcgcagaacgcatgggctggcacctccccggcttcgacgacagcgcctggacggccgagaactcaactgcatccacctcggcactgagcttcaccggcgcaaccgtccgcttcttccgcaccgtcgtccccctcgatatccctgctggtctggacgtctccgtctccttcgtgctctcgaccccatcgaatgcgcccaagggataccgcgcacagctgttcgtcaatgggtaccagtatggtcggtacaacccacacatcggcaatcaggtggtgttccctgttccgccgggtattctcgattaccagggagataacacgatcgggttggcggtctgggcgcagacggaagagggggcgagtatccaggtggactggaaggtgaattacgtggcggatagctcgttgagtgtcgctggatttgggaaaggcttgaggccgggttggaccgaggagcggttgaagtttacctag

SEQ ID NO: 78 - protein, 1014 aa, Aspergillus lentulus
MAHIYQLLLLLLSNLWFATAAQNQSETEWPLHDNGLSKVVQWDHYSFHVNGQRIFVFSGEFHYWRIPVPELWRDVLEKVKATGFTAFAFYSSWAYHAPNNHTVDFSTGARDITPIFELAKELGMYMIVRPGPYVNAEASAGGFPLWLTTGEYGSLRNDDPRYTAAWTPYFANMSQITSKYQVTDGHNTLVYQIENEYGQQWIGDPKDRKPNKTAVAYMELLEASARENGITVPLTSNDPNMNSKSWGSDWSNAGGNVDVAGLDSYPSCWTCDVSQCTSTNGEYVPYKVIDYYDYFQEVQPTLPSFMPEFQGGSYNPWAGPEGGCPQDTGAEFANLFYRWNIGQRVTAMSLYMLYGGTNWGAIAAPVTATSYDYSAPISEDRSIGAKYSETKLLALFTRTAKDLTMTEAIGNGTQYTTNTAVRAFELRNPQTNAGFYVTFHNDTTVGGNQAFKLHVNTSVGALTVPKNEGVIQLNGHQSKIIVTDFTLGKRTLLYSTAEVLTYAVFEDRPTLVLWVPTGESGEFAIKGAKSGKVENGDGCSGIKFESEKNYLVVNFSQAKGLSVLRLDNGVRVVLLDKAAAYRFWAPALTNDPVVQEAETVLVHGPYLVRSASVSKSTLALRGDSVEKTTLEIFAPHSVREITWNGKQVKTSQTSYGSLKATLAAPPTIKLPALTSWRSNDSLPERLPSYDDSGPAWIEANHMTTSNPSKPATLPVLYADEYGFHNGVRLWRGYFNGSASGVYLNIQGGSAFGWSAWLNGHFLDSHLGDATTSQANKTLPFPPSLLNPTENVLLIVHDDTGHDQTTGALNPRGILAARLLSNDSSSPAPEFTRWRLAGTAGGESNLDPIRGVFNEDGLFAERMGWHLPGFDDSAWTAENSTASTSALSFTGATVRFFRTVVPLDIPAGLDVSVSFVLSTPSNAPKGYRAQLFVNGYQYGRYNPHIGNQVVFPVPPGILDYQGDNTIGLAVWAQTEEGASIQVDWKVNYVADSSLSVAGFGKGLRPGWTEERLKFT

SEQ ID NO: 79 - protein, 994 aa, Aspergillus lentulus
  mat_peptide (1)..(994)
AQNQSETEWPLHDNGLSKVVQWDHYSFHVNGQRIFVFSGEFHYWRIPVPELWRDVLEKVKATGFTAFAFYSSWAYHAPNNHTVDFSTGARDITPIFELAKELGMYMIVRPGPYVNAEASAGGFPLWLTTGEYGSLRNDDPRYTAAWTPYFANMSQITSKYQVTDGHNTLVYQIENEYGQQWIGDPKDRKPNKTAVAYMELLEASARENGITVPLTSNDPNMNSKSWGSDWSNAGGNVDVAGLDSYPSCWTCDVSQCTSTNGEYVPYKVIDYYDYFQEVQPTLPSFMPEFQGGSYNPWAGPEGGCPQDTGAEFANLFYRWNIGQRVTAMSLYMLYGGTNWGAIAAPVTATSYDYSAPISEDRSIGAKYSETKLLALFTRTAKDLTMTEAIGNGTQYTTNTAVRAFELRNPQTNAGFYVTFHNDTTVGGNQAFKLHVNTSVGALTVPKNEGVIQLNGHQSKIIVTDFTLGKRTLLYSTAEVLTYAVFEDRPTLVLWVPTGESGEFAIKGAKSGKVENGDGCSGIKFESEKNYLVVNFSQAKGLSVLRLDNGVRVVLLDKAAAYRFWAPALTNDPVVQEAETVLVHGPYLVRSASVSKSTLALRGDSVEKTTLEIFAPHSVREITWNGKQVKTSQTSYGSLKATLAAPPTIKLPALTSWRSNDSLPERLPSYDDSGPAWIEANHMTTSNPSKPATLPVLYADEYGFHNGVRLWRGYFNGSASGVYLNIQGGSAFGWSAWLNGHFLDSHLGDATTSQANKTLPFPPSLLNPTENVLLIVHDDTGHDQTTGALNPRGILAARLLSNDSSSPAPEFTRWRLAGTAGGESNLDPIRGVFNEDGLFAERMGWHLPGFDDSAWTAENSTASTSALSFTGATVRFFRTVVPLDIPAGLDVSVSFVLSTPSNAPKGYRAQLFVNGYQYGRYNPHIGNQVVFPVPPGILDYQGDNTIGLAVWAQTEEGASIQVDWKVNYVADSSLSVAGFGKGLRPGWTEERLKFT

SEQ ID NO: 80 - protein, 5 aa, Artificial Sequence
  SEQ ID NO: 80 is the conserved motif Y[Y/F][D/Q][Y/H/W]F.
  MISC_FEATURE (2)..(2): The amino acid in position 2 of the conserved motif is either phenylalanine (F) or tyrosine (Y).
  MISC_FEATURE (3)..(3): The amino acid in position 3 of the conserved motif is either aspartic acid (D) or glutamine (Q).
  MISC_FEATURE (4)..(4): The amino acid in position 4 of the conserved motif is either phenylalanine (F), tyrosine (Y) or tryptophan (W).
YXXXF

SEQ ID NO: 81 - protein, 6 aa, Artificial Sequence
  SEQ ID NO: 81 is the conserved motif K[Y/F][Y/S]ETK.
  MISC_FEATURE (2)..(2): The amino acid in position 2 of the conserved motif is either phenylalanine (F) or tyrosine (Y).
  MISC_FEATURE (3)..(3): The amino acid in position 3 of the conserved motif is either serine (S) or tyrosine (Y).
KXXETK

SEQ ID NO: 82 - protein, 1013 aa, Penicillium chrysogenum
MTRILNCLLVLLACLGVSSKAEDQAVTQWPLQDNGLNTVVQWDHYSFQINGQRIFIFSGEFHYWRIPVPALWRDILEKIKAAGFTAFAFYSSWAYHAPNNATVDFTTGARDITPIFELAKELGMYIIVRPGPYVNAEANAGGFPLWVTTGDYGTLRNDDTRYTNAWTPYFTEVTEITSRYQVTDGHYSIVYQIENEYGNQWLGDPTLRVPNETAIAYMELLKANARDNGITLPLTVNDPNMKTHSWGKDWSDAGGNVDAAGLDSYPSCWTCDISQCTSTNGAYVPFQVLEYHDYFQESQPSMPAFMPEFQGGSYNPWGGPEGGCPGDIGDDFANLFYRWNIGQRVTAMSLYMMFGGQNPGAMAAPVTASSYDYSAPISEDRSIWSKYHETKLLALFTRSAKDLTMTELMGNGTQYTDNPAVRAYELRNPETNSAFYATFHSNTSISTNEPFHLKVNTSAGVLTVPKYASTIRLNGHQSKIIVTDFTFGSKSLLYSTAEVLTYAVFDKKPTLVLWVPTGESGEFSIKGAKKGSIKKCQGCSRVKFIKEHGGLTTSLTQSAGMTVLEFDDGVRVILLDRTSAYDFWAPALTNDPFVPETESVLIQGPYLVRDAKLSGSKLAITGDVVNATTLDVFAPKGVKSVTWNGKKVDTHSTEYGSLKGSLDAPQSIKLPALASWKSKDSLPERFADYDDSGAAWVDANHMTTLNPRTPTSLPVLYADQYGFHNGVRLWRGYFNGTATGAFINVQGGSAFGWSAWLNGEFLASHLGNATTSQANLSLSFTDATLHTDTPNVLLIVHDDTGHDQTTGALNPRGIMDAKLLGSDSGFTHWRLAGTAGGESDLDPVRGVYNEDGLFAERVGWHLPGFDDSDWGEEASAKDSTTSVLSFEGATVRFFRTTCPLDIPAHTDVSISFVLSTPAGATTEYRAQLFVNGYQYGRYNPYIGNQVVYPVPVGILDYKGENTIGVAVWAQSEEGASIGIDWRVNYLADSSLDVASWDTKDLRPGWTEERVKYA

SEQ ID NO: 83 - protein, 352 aa, Penicillium chrysogenum
MLPHLLLAAAQLFASSSAALTYNGADISSLLVEEGKGVSYKNLAGTPEKLETILSASGVNSVRQRIWVNPSDGSYDLDYNVKLAKRVQAQGMGTYLDLHYSDTWADPKSQTTPSGWSTTDIGILAGQVYDYTLDVCNTFAANKIDVDIVSIGNEIRNGLLWPLGGTSNYNNIARLLHSAAWGVKDSKLATTPKIMIHLDNGWDSGAQSYFYDQVLAPGSGLVSTDFDYIGVSYYPFYNADATLAALKTSLTNLHSKYKKETLVVETNWPFSCPNPEYAFPTDLKDIPFSVEGQQTFLQRLAKAVEEVGGLGIYYWEPAWVDNAGLGSSCDDNLFFAWSNDQARASLDTLGGL

SEQ ID NO: 84 - protein, 1007 aa, Aspergillus niger
MKLSSACAIALLAAQAAGASIKHRINGFTLTEHSDPAKRELLQKYVTWDDKSLFINGERIMIFSGEFHPFRLPVKELQLDIFQKVKALGFNCVSFYVDWALVEGKPGEYRADGIFDLEPFFDAASEAGIYLLARPGPYINAESSGGGFPGWLQRVNGTLRSSDKAYLDATDNYVSHVAATIAKYQITNGGPIILYQPENEYTSGCCGVEFPDPVYMQYVEDQARNAGVVIPLINNDASASGNNAPGTGKGAVDIYGHDSYPLGFDCANPTVWPSGDLPTNFRTLHLEQSPTTPYAIVEFQGGSYDPWGGPGFAACSELLNNEFERVFYKNDFSFQIAIMNLYMIFGGTNWGNLGYPNGYTSYDYGSAVTESRNITREKYSELKLLGNFAKVSPGYLTASPGNLTTSGYADTTDLTVTPLLGNSTGSFFVVRHSDYSSEESTSYKLRLPTSAGSVTIPQLGGTLTLNGRDSKIHVTDYNVSGTNIIYSTAEVFTWKKFADGKVLVLYGGAGEHHELAISTKSNVTVIEGSESGISSKQTSSSVVVGWDVSTTRRIIQVGDLKILLLDRNSAYNYWVPQLATDGTSPGFSTPEKVASSIIVKAGYLVRTAYLKGSGLYLTADFNATTSVEVIGVPSTAKNLFINGDKTSHTVDKNGIWSATVDYNAPDISLPSLKDLDWKYVDTLPEIQSSYDDSLWPAADLKQTKNTLRSLTTPTSLYSSDYGFHTGYLLYRGHFTATGNESTFAIDTQGGSAFGSSVWLNGTYLGSWTGLYANSDYNATYNLPQLQAGKTYVITVVIDNMGLEENWTVGEDLMKTPRGILNFLLAGRPSSAISWKLTGNLGGEDYEDKVRGPLNEGGLYAERQGFHQPEPPSQNWKSSSPLEGLSEAGIGFYSASFDLDLPKGWDVPLFLNIGNSTTPSPYRVQVYVNGYQYAKYISNIGPQTSFPVPEGILNYRGTNWLAVTLWALDSAGGKLESLELSYTTPVLTALGEVESVDQPKYKKRKGAY

SEQ ID NO: 85 - protein, 350 aa, Aspergillus niger
MIYPLLLSALPLLSSAALTYRGADISSLLIEEDAGISYKNLNGETQALEDILVNNGVNSIRQRVWVDPSDGSYDLDYNLKLAKRVQAAGMSIYLDLHLSDTWADPSDQTTPTGWSTTDIDTLTWQLYNYTLDVCNTFAENDIDIEIVSIGNEISSGLLWPLGKTSNYDNIAKLLHSGAWGVKDSNQATTPKIMIHLDNGWDWEEQEYFYKTVLATGSLLSTDFDLMGVSYYPFYNSEATLSALQTSLTNMQSNYDKSVVVVETNWPVSCPDPEYSFPSDLSSIPFSAAGQEEFLEKLAEVVEGVTDGLGIYYWEPAWVDNAALASSCADNLMVDIDTDEVLESVTVFEDL